European Patent Specification EP 3 458 105 B1, published January 17, 2024. Title: POLYNUCLEOTIDES ENCODING GALACTOSE-1-PHOSPHATE URIDYLYLTRANSFERASE FOR THE TREATMENT OF GALACTOSEMIA TYPE 1. Applicant: MODERNATX, INC. The sequence listing filed with the application follows.

SEQUENCE LISTING (173 sequences)

SEQ ID NO: 1 - protein, 379 aa, Artificial Sequence
  wild-type isoform 1 of human GALT
MSRSGTDPQQRQQASEADAAAATFRANDHQHIRYNPLQDEWVLVSAHRMKRPWQGQVEPQLLKTVPRHDPLNPLCPGAIRANGEVNPQYDSTFLFDNDFPALQPDAPSPGPSDHPLFQAKSARGVCKVMCFHPWSDVTLPLMSVPEIRAVVDAWASVTEELGAQYPWVQIFENKGAMMGCSNPHPHCQVWASSFLPDIAQREERSQQAYKSQHGEPLLMEYSRQELLRKERLVLTSEHWLVLVPFWATWPYQTLLLPRRHVRRLPELTPAERDDLASIMKKLLTKYDNLFETSFPYSMGWHGAPTGSEAGANWNHWQLHAHYYPPLLRSATVRKFMVGYEMLAQAQRDLTPEQAAERLRALPEVHYHLGQKDRETATIA

SEQ ID NO: 2 - DNA, 1137 bp, Artificial Sequence
  nucleotide sequence of wild type PBGD, isoform 1
atgtcgcgcagtggaaccgatcctcagcaacgccagcaggcgtcagaggcggacgccgcagcagcaaccttccgggcaaacgaccatcagcatatccgctacaacccgctgcaggatgagtgggtgctggtgtcagctcaccgcatgaagcggccctggcagggtcaagtggagccccagcttctgaagacagtgccccgccatgaccctctcaaccctctgtgtcctggggccatccgagccaacggagaggtgaatccccagtacgatagcaccttcctgtttgacaacgacttcccagctctgcagcctgatgcccccagtccaggacccagtgatcatccccttttccaagcaaagtctgctcgaggagtctgtaaggtcatgtgcttccacccctggtcggatgtaacgctgccactcatgtcggtccctgagatccgggctgttgttgatgcatgggcctcagtcacagaggagctgggtgcccagtacccttgggtgcagatctttgaaaacaaaggtgccatgatgggctgttctaacccccacccccactgccaggtatgggccagcagtttcctgccagatattgcccagcgtgaggagcgatctcagcaggcctataagagtcagcatggagagcccctgctaatggagtacagccgccaggagctactcaggaaggaacgtctggtcctaaccagtgagcactggttagtactggtccccttctgggcaacatggccctaccagacactgctgctgccccgtcggcatgtgcggcggctacctgagctgacccctgctgagcgtgatgatctagcctccatcatgaagaagctcttgaccaagtatgacaacctctttgagacgtcctttccctactccatgggctggcatggggctcccacaggatcagaggctggggccaactggaaccattggcagctgcacgctcattactaccctccgctcctgcgctctgccactgtccggaaattcatggttggctacgaaatgcttgctcaggctcagagggacctcacccctgagcaggctgcagagagactaagggcacttcctgaggttcattaccacctggggcagaaggacagggagacagcaaccatcgcc

SEQ ID NO: 3 - protein, 270 aa, Artificial Sequence
  wild-type isoform 2 of human GALT
MTLSTLCVLGPSEPTESKVMCFHPWSDVTLPLMSVPEIRAVVDAWASVTEELGAQYPWVQIFENKGAMMGCSNPHPHCQVWASSFLPDIAQREERSQQAYKSQHGEPLLMEYSRQELLRKERLVLTSEHWLVLVPFWATWPYQTLLLPRRHVRRLPELTPAERDDLASIMKKLLTKYDNLFETSFPYSMGWHGAPTGSEAGANWNHWQLHAHYYPPLLRSATVRKFMVGYEMLAQAQRDLTPEQAAERLRALPEVHYHLGQKDRETATIA

SEQ ID NO: 4 - DNA, 810 bp, Artificial Sequence
  wild type isoform
atgaccctctcaaccctctgtgtcctggggccatccgagccaacggagagtaaggtcatgtgcttccacccctggtcggatgtaacgctgccactcatgtcggtccctgagatccgggctgttgttgatgcatgggcctcagtcacagaggagctgggtgcccagtacccttgggtgcagatctttgaaaacaaaggtgccatgatgggctgttctaacccccacccccactgccaggtatgggccagcagtttcctgccagatattgcccagcgtgaggagcgatctcagcaggcctataagagtcagcatggagagcccctgctaatggagtacagccgccaggagctactcaggaaggaacgtctggtcctaaccagtgagcactggttagtactggtccccttctgggcaacatggccctaccagacactgctgctgccccgtcggcatgtgcggcggctacctgagctgacccctgctgagcgtgatgatctagcctccatcatgaagaagctcttgaccaagtatgacaacctctttgagacgtcctttccctactccatgggctggcatggggctcccacaggatcagaggctggggccaactggaaccattggcagctgcacgctcattactaccctccgctcctgcgctctgccactgtccggaaattcatggttggctacgaaatgcttgctcaggctcagagggacctcacccctgagcaggctgcagagagactaagggcacttcctgaggttcattaccacctggggcagaaggacagggagacagcaaccatcgcc

SEQ ID NO: 5 - RNA, 1137 nt, Artificial Sequence
  GALT-CO01
augagcagguccgggaccgauccccagcagaggcagcaggccuccgaggcggacgccgccgccgccaccuuucgcgccaacgaccaccagcauaucagguacaaccccuugcaagacgaguggguccuagugagcgcccacaggaugaagcggcccuggcagggccagguggagccccagcugcugaagaccgugccucgccacgacccccugaacccccugugccccggggccaucagggccaacggugaggugaacccacaauacgauucgaccuuccuauucgacaacgauuuccccgcccuccagcccgaugcccccagccccggcccguccgaccauccgcuguuccaggccaaguccgccaggggaguguguaaggugaugugcuuucaccccugguccgaugugacccucccgcugaugagcgugcccgagaucagggcaguggucgacgccugggcgagcgugaccgaagagcucggugcccaguacccgugggugcagaucuucgagaauaagggcgccaugaugggcugcagcaacccccauccccacugccaagugugggcaagcagcuuccugcccgacaucgcccagagggaggagcgcucccagcaggccuacaaaagccagcacggcgaaccccuucugauggaguacagccggcaggagcugcucaggaaagagaggcuggugcugacaagcgagcacuggcucgugcuggugccguucugggccaccuggcccuaccagacccugcugcugcccaggaggcacgugaggcgucuucccgaacucacgcccgccgagagggaugaucuggccuccaucaugaagaagcugcugaccaaauacgacaaucucuucgagaccuccuuccccuacagcaugggauggcacggcgccccgaccggcuccgaggccggcgccaauuggaaccacuggcagcuccacgcccacuacuaccccccccuccugagguccgccaccgugcguaaguucaugguaggcuaugagaugcuggcccaggcccagcgggaccugaccccggagcaggccgccgagcggcugcgggcccuccccgagguccacuaucaccucggccagaaagacagggagaccgccaccaucgcc

SEQ ID NO: 6 - RNA, 1137 nt, Artificial Sequence
  GALT-CO02
augucccgaagcggcaccgauccgcagcagcggcagcaggcaucagaggccgacgccgccgccgccaccuuucgugccaacgaccaccagcacauuagguacaauccccugcaagacgagugggugcuggugagcgcccaccggaugaaaaggcccuggcagggccaggucgagccccagcuacucaagaccguccccaggcacgacccccugaacccccucugccccggcgcgauccgggccaauggcgaggugaacccccaguacgauuccaccuuccuguucgacaacgacuuccccgcccugcagcccgaugccccgagccccggccccagcgaccacccccuguuccaggccaaauccgccagaggugugugcaaggugaugugcuuccaccccuggagcgacgugacccugccccucaugagcguccccgagauccgcgcagugguggacgccugggcguccgugaccgaggagcugggggcccaguaccccugggugcagaucuuugagaauaagggcgccaugaugggcuguagcaacccccacccccacugucaggugugggccagcagcuuccugcccgacaucgcccagagggaagagcgcagccagcaggccuauaagagccagcauggggagccccugcucauggaauacucccgucaggagcugcugcggaaggagaggcuggugcugacuagcgagcauuggcuggugcuggugcccuucugggccaccuggccuuaccagacccugcugcucccccggaggcacgugcgaaggcugcccgagcugacccccgccgagcgcgacgaccuggccucaaucaugaagaagcugcugaccaaguacgacaaccuuuucgagaccuccuucccguauagcaugggcuggcacggcgcccccaccggcagcgaggccggcgccaacuggaaccacuggcagcugcacgcgcacuacuacccuccccugcucaggagcgccaccgugcggaaguucauggugggcuacgaaaugcuggcccaagcgcagcgcgaccucacccccgagcaggccgccgaaaggcuccgugcccugccagaggugcacuaccaccugggucaaaaggaucgggagaccgccaccaucgcc

SEQ ID NO: 7 - RNA, 1137 nt, Artificial Sequence
  GALT-CO03
augagcaggagcgguaccgacccccagcaacggcagcaggccuccgaggccgacgcagccgccgccaccuuccgcgccaacgaccaucagcauauccgcuacaacccccugcaggacgagugggugcugguguccgcccacaggaugaagcggcccuggcagggccagguggagccccagcugcugaaaaccgugccgcgacacgacccccuuaacccccucugucccggugccauccgcgccaacggcgaggugaacccacaguacgacagcacauuccuguuugacaacgacuuucccgcucuccagcccgacgcccccagccccggccccagcgaccauccccucuuccaggccaagagugcgcggggcgugugcaaggugauguguuuccaccccugguccgacgugacccugccucugaugagcgugcccgagaucagggccguggucgacgccugggccucggugaccgaggagcugggcgcccaauaccccuggguccagaucuucgaaaacaagggcgccaugaugggcugcagcaacccccacccucacugucaggugugggccuccuccuuccuccccgacaucgcccagagggaagaaaggagccagcaggccuacaagucacaacacggcgagccgcugcugauggaguacuccaggcaggagcugcugaggaaggagcggcuggugcugaccagcgagcacuggcugguccuggugcccuucugggccaccuggccguaccagaccuugcugcugcccaggaggcaugugaggaggcugccagagcucacccccgccgaacgggacgaccuggccucuaucaugaagaagcugcugaccaaguaugacaaccuguucgaaacgagcuucccauacagcaugggcuggcacggggcacccaccggcagcgaggccggcgccaacuggaaccacuggcagcugcacgcccauuacuacccgccccugcugcggagcgccaccguccggaaguucauggugggcuacgagaugcuggcacaggcgcagagggaccugacccccgagcaggccgcagagcggcuccgggcccugcccgaggugcacuaccaccucggccagaaggauagggagaccgccaccaucgcc

SEQ ID NO: 8 - RNA, 1137 nt, Artificial Sequence
  GALT-CO04
augagccggagcggcaccgacccccaacagcgccagcaggccuccgaagccgacgccgccgccgccaccuuccgcgccaacgaccaccagcauauccgguauaacccccugcaggacgagugggugcuggugagcgcccacagaaugaagaggcccuggcagggccagguugaaccccaacugcugaagaccgugcccaggcacgacccccugaacccgcugugcccgggagccaucagggccaacggcgaggucaacccccaguacgauagcacguuccuguuugacaaugacuucccagcccugcaacccgaugccccaucccccgggccauccgaccacccccuguuccaggccaaguccgcccgaggcgucugcaaggugaugugcuuucaccccuggagcgacgugacccugccccugaugagcgugccggagauccgcgccgugguggacgccugggcguccgugaccgaagaacugggcgcccaauaccccugggugcagaucuucgagaacaagggcgccaugaugggaugcuccaacccccacccccauugccaggugugggccagcagcuuccugcccgacaucgcccagagggaagagaggagccagcaggccuacaagucacagcacggugagccccugcucauggaauacagcaggcaggagcugcugcgcaaggagcgccuggugcucaccagcgagcauuggcuggugcuggugcccuucugggccacauggcccuaccagacccugcugcuccccaggaggcacgugaggcggcugcccgagcucacgccggcggagagggacgaccuggcgagcaucaugaagaagcugcugaccaaauacgacaaccucuuugagaccagcuuucccuauagcaugggcuggcacggcgcccccaccgggagcgaagccggcgccaacuggaaccauuggcagcugcacgcccacuacuaccccccccugcugagaagcgccaccgugcgaaaguucauggugggcuaugagaugcuggcccaagcccagcgcgaccugaccccggaacaggccgccgagagacugcgcgcccugcccgagguccacuaccaccucggacagaaggacagggagaccgccaccauugcc

SEQ ID NO: 9 - RNA, 1137 nt, Artificial Sequence
  GALT-CO05
auguccagguccggcaccgauccccaacaaaggcagcaggccuccgaggccgacgccgccgccgcgaccuucagggccaacgaccaccagcacaucagguauaacccccuccaggacgagugggugcuggugagcgcccacaggaugaagcgccccuggcagggccaggucgaaccccagcuccugaagaccgugccccgccacgacccccugaacccccucugcccgggcgccauccgggccaacggugaggugaacccccaguacgacagcacguuucuguuugacaacgacuuccccgccuugcagcccgacgcccccagccccggccccagcgaccauccccuguuucaagccaaaagcgcacggggcgugugcaaggugaugugcuuccacccguggagcgacgugacacugccgcugaugucggugccggagaucagggccgucguggacgcgugggccuccgugaccgaggagcugggggcccaguaccccugggugcagaucuucgagaacaagggagccaugaugggcugcagcaauccccacccccacugccaggucugggccagcagcuuucugcccgacaucgcccaacgggaggaacgcagccaacaggccuacaagagccagcauggcgaaccgcugcugauggaguacagccgccaggagcugcugcggaaggaaaggcuggugcugacauccgaacacuggcuggugcuggugcccuucugggccaccuggcccuaccagacccugcugcugcccaggcgccacgugaggaggcugcccgagcugacccccgccgagagggacgaucuggcgagcaucaugaagaagcuccucaccaaguacgacaaccuuuucgagaccagcuuucccuacagcauggguuggcacggcgcccccaccggcagcgaggccggugccaacuggaaccacuggcaacugcacgcgcacuacuaccccccccugcugagguccgccaccgugcguaaguucauggucggauaugaaaugcuggcccaagcgcagagggaccucacccccgagcaggccgccgagcgccugagggcccugcccgaggugcauuaccaccuggggcagaaggacagggagacggccaccaucgcc

SEQ ID NO: 10 - RNA, 1137 nt, Artificial Sequence
  GALT-CO06
augagcaggagcgguacggacccgcagcaaaggcagcaggccagcgaggccgacgccgccgccgccaccuuccgggccaacgaccaccaacacauccgguacaacccccugcaggacgagugggugcuggugagcgcacaccggaugaagaggcccuggcagggccagguggagccccaacugcugaagaccgugcccaggcacgacccgcugaauccccugugucccggugccauuagggccaauggggaggugaacccgcaguacgauagcacguuccuguucgauaaugacuuccccgcccugcagccggacgccccgucccccggccccagcgaccacccgcucuuucaggccaagagcgccaggggcgugugcaaggugauguguuuucaccccuggagcgacgugacccugccccugauguccgugcccgagauccgcgccgugguggacgcaugggccagcgugaccgaggaacugggggcccaguaccccugggugcagauauucgagaacaaaggcgccaugaugggcugcagcaacccccacccccacugccaggugugggccucgucguuucuccccgauaucgcccaaagggaggagaggucccagcaggccuauaagagccagcauggcgaaccccugcugauggaguacagcaggcaggagcugcugcggaaagaaaggcugguccugaccagcgagcauuggcuggugcuggugcccuucugggccaccuggcccuaccagacgcugcugcugcccaggaggcacgucaggcgccugcccgaacugacccccgccgagcgcgaugaccucgcuagcauaaugaagaagcugcugaccaaguacgacaaccuguuugaaaccagcuucccguacucaaugggcuggcauggcgccccgacggguagcgaggcgggcgccaacuggaaccacuggcagcugcacgcccacuacuaccccccccugcucaggagcgccaccgugaggaaguuuauggugggcuacgagaugcuggcccaggcgcagagggaccugacccccgagcaggcggccgagaggcugcgagcccugcccgagguccauuaccaccugggccagaaggacagggaaacggccacgauugcc

SEQ ID NO: 11 - RNA, 1137 nt, Artificial Sequence
  GALT-CO07
augagcaggagcggcaccgauccccagcagaggcagcaggccagcgaggccgacgccgccgccgccacguucagggccaacgaucaccagcacaucagguacaacccacugcaggacgagugggugcuggugagcgcgcaucggaugaaacgccccuggcagggccaggucgagccgcaacuccugaagaccgugccaaggcacgacccccugaacccccuaugccccggcgcgaucagggccaacggcgaggugaacccccaguacgauucgaccuuucucuucgauaacgacuuccccgcccugcaacccgacgcccccagccccgggcccuccgaccacccgcucuuccaggccaaguccgcccgcggcgucuguaaggugaugugcuuccaccccuggucggacgugacccucccgcucaugagcguccccgaaauccgagccgugguggacgccugggccucggugacggaggagcugggcgcccaauaccccugggugcagauuuuugagaacaagggggcgaugaugggcugcagcaacccccacccacacugccaggucugggccaguagcuuucugcccgauaucgcgcaaagggaagagaggagccagcaggcauauaaaagccagcauggcgagccccugcuuauggaguacuccaggcaggagcugcugaggaaggagaggcucgugcuaaccagcgagcauuggcugguccuggugcccuucugggccaccuggccauaccagaccuugcugcugccccgccggcacguccgcagacugcccgagcucacgcccgccgagagggaugaucuggccagcaucaugaagaagcugcucaccaaauacgauaaccuguucgagaccagcuucccguacagcaugggguggcacggcgcgcccaccggcagcgaggccggcgccaauuggaaucacuggcagcugcaugcccacuacuaccccccccuccugcggucggccaccgugaggaaauucauggugggcuaugagaugcuggcccaggcgcagagggaccugacccccgaacaggccgccgaacgacugagggcccuccccgaggugcacuaucaccucgggcaaaaagacagggagaccgccaccaucgcc

SEQ ID NO: 12 - RNA, 1137 nt, Artificial Sequence
  GALT-CO08
augagccggagcgggaccgacccacagcagcggcagcaggccagcgaggcggacgccgccgccgccacauuccgcgccaacgaucaccagcacauccgcuauaauccccugcaggacgaguggguccuggugagcgcucacaggaugaagcgucccuggcaaggccagguggagccccagcugcugaaaaccgugccgaggcacgacccgcuaaacccguuaugucccggcgccauccgagccaacggcgaagugaauccgcaguacgacagcaccuuccucuuugacaacgacuuccccgcgcugcagcccgacgcccccucccccggccccagcgaccacccgcuguuccaggccaagagcgcccgaggcgugugcaaagucaugugcuuccaccccuggagcgacgugacucugccccugaugagcgugcccgagauccgcgccgugguggacgccugggccagcgucacggaagagcugggcgcgcaauaccccugggugcagaucuucgagaacaagggggccaugauggggugcagcaauccccacccccacugccaggugugggccagcagcuuccugccggacaucgcucagcgggaggagaggagccaacaggccuacaaaagccaacacggggagccccugcugauggaguacagcaggcaggagcugcucaggaaagagcggcuggugcugaccuccgagcauuggcuggugcucguacccuucugggccaccuggcccuaccagacucugcugcugccgcgccggcacgugcgaaggcuccccgagcuuaccccggccgaacgggacgaccucgccagcaucaugaaaaagcugcugaccaaguacgauaaucuguucgaaaccagcuuuccauacaguaugggcuggcacggcgcccccaccgguagcgaggccggcgcgaacuggaaccauuggcagcugcacgcccacuacuacccuccccuccugcguuccgccaccgugaggaaguucauggugggcuacgagaugcuggcccaggcccaacgggaucugacccccgagcaggccgccgagcggcuccgggcccugcccgaggugcacuaccaccugggccagaaggaccgggagaccgccacgaucgcc

SEQ ID NO: 13 - RNA, 1137 nt, Artificial Sequence
  GALT-CO09
augagccgguccggcaccgacccccagcagaggcagcaggccagcgaggccgacgccgccgccgcgaccuuucgggccaacgaccaccagcacaucagauacaacccgcuccaggacgagugggugcuggugagcgcccacaggaugaagaggccguggcaggggcaaguggaaccccagcuacugaagaccgugcccaggcacgauccccugaacccccugugcccgggagccauccgggcaaacggggaggugaacccccaguacgacagcaccuuucuguuugacaacgacuucccggcccuccagccggacgcccccucccccggcccgagcgaccacccccuguuccaggccaaauccgccaggggcgugugcaaggugauguguuuccacccaugguccgaugugacgcugccccugaugagcguccccgagaucagggccgugguggaugccugggccagcgugaccgaggagcugggggcccaguaccccugggugcaaaucuuugagaacaagggggccaugaugggcugcagcaacccccacccccacugucaggugugggccuccagcuuucuccccgacauugcccagagggaggagcguagccagcaggccuacaagagccagcacggggagccccugcugauggaguacucccggcaagagcuccuccggaaggagaggcuugugcugacgucggagcauuggcugguacuggugcccuucugggccaccuggcccuaccagacucugcugcucccccggcggcacgugcguaggcugcccgagcugacccccgccgagcgggacgaccucgccagcaucaugaagaagcuccugacaaaguacgacaaucuguucgagacuuccuuccccuacuccaugggguggcacggcgcccccaccggcagcgaggccggggccaacuggaaccacuggcaacugcaugcccacuauuaccccccccuucugcguagcgcgaccgugcggaaguucauggucggcuacgagaugcuggcccaggcccagagggaccugacgcccgaacaggccgccgagcggcugagggcccugcccgaggugcacuaccaccuggggcagaaagaccgcgagaccgccacuaucgcc

SEQ ID NO: 14 - RNA, 1137 nt, Artificial Sequence
  GALT-CO10
augagccggagcggcaccgacccccaacagaggcagcaagccagcgaggccgacgccgccgcggccaccuuucgagccaacgaccaccagcacauccgguacaacccgcugcaggacgaguggguucuggucucggcccaccgaaugaagcgccccuggcagggccaggucgagccgcagcugcugaagacgguucccaggcacgacccccucaacccccugugccccggcgccauccgggcaaauggggaggugaauccccaguacgacagcaccuuccuguucgacaacgauuuccccgcccugcagcccgacgccccauccccaggacccuccgaccacccccucuuucaggccaaauccgcgcgaggcgugugcaaggucaugugcuuucaccccugguccgaugugacacugccgcuuaugucaguccccgagauccgggcggugguggaugccugggccagcgugaccgaggagcucggcgcccaauaccccugggugcagaucuucgaaaacaaaggcgccaugaugggcugcuccaauccccacccccacugccaggugugggcuagcuccuuccugccggacaucgcgcagcgggaagagcggucccagcaggccuauaagagucagcacggcgagccccugcugauggaauacagcaggcaggagcugcugcggaaagagcgccuggugcugaccagcgaacacuggcugguacugguccccuuuugggccacuuggccguaccaaacccuccugcuccccaggcggcacgugcgcaggcugccugagcugaccccggccgagagggacgaccuggcaucaaucaugaagaagcugcugacgaaguacgacaaucucuucgaaaccagcuuccccuacagcaugggguggcauggcgccccgacggggagcgaggccggcgccaacuggaaucauuggcagcugcacgcccacuauuaccccccccugcugaggagcgccaccgugaggaaauucauggucggcuacgaaaugcuggcccaggcccagcgggaucugacgccugagcaagccgccgagaggcugcgggcccugccagaggugcacuaccaucucggccagaaagaccgcgagaccgcgaccauagcc

SEQ ID NO: 15 - RNA, 1137 nt, Artificial Sequence
  GALT-CO11
auguccagguccggcacggacccccagcagcgccagcaagccagcgaggccgacgccgccgcggcgaccuuccgggccaacgaccaccagcacaucagguacaacccgcugcaggacgagugggugcuggugagcgcccacaggaugaagcggcccuggcagggccagguagagccccaacugcugaagaccgugcccaggcacgacccgcugaacccccugugccccggcgccauccgcgccaacggcgaggugaacccacaguacgauagcaccuuucucuucgacaaugauuuccccgcccugcagcccgacgccccaagccccggccccucagaccacccccuguuccaagccaagagcgcgaggggcguguguaaggugaugugcuuccaccccuggagcgaugugacgcugccccugaugagcgucccggagaucagggccguggucgacgccugggcguccgugaccgaggagcugggggcccaguaccccuggguccagaucuucgagaacaagggcgccaugaugggcugcagcaauccccacccccauugccaggugugggccucuagcuuccugcccgacaucgcccagagggaggagaggagccagcaagccuauaagagccagcacggggagccgcugcugauggaguacucccgccaggagcuccucaggaaggagcggcuggugcugacaagcgagcacuggcuggugcucgugcccuuuugggcaacauggcccuaccagacccugcugcugccccggcggcacgugaggaggcugcccgagcugacccccgccgaaagggaugaucuggccuccaucaugaagaagcuccugaccaaguacgacaaccucuucgaaacaucguuccccuacagcaugggcuggcacggugccccgacaggcuccgaagccggcgccaacuggaaccacuggcagcugcacgcgcacuacuaccccccccugcugaggagugcuaccgugcgaaaguuuauggugggcuacgagaugcuggcgcaggcccagagggaccugacacccgaacaggccgccgagcggcugcgggcccugcccgagguccacuaccaccucggccagaaggaccgggagaccgccacgauagcc

SEQ ID NO: 16 - RNA, 1137 nt, Artificial Sequence
  GALT-CO12
augagcaggagcggcaccgacccccagcagcggcagcaagcguccgaggccgacgccgccgccgccacauuccgugccaacgaucaccaacacauacgguacaacccgcugcaggacgagugggugcuggugagcgcccaccgcaugaagaggcccuggcagggccagguggagccccagcugcugaagaccgugccucggcacgacccccugaacccccucugccccggggccaucagggccaacggcgaggugaacccgcaauacgacagcaccuuccuguucgacaacgacuuccccgcccugcaacccgacgcacccagccccggcccgagcgaucacccgcucuuccaggcgaagagcgccaggggcgugugcaaggugaugugcuuccauccguggagcgaugugacccugccccugaugagcgucccugaaaucagggccgugguggacgccugggccucugugaccgaggagcucggggcccaguauccgugggugcagaucuucgagaacaagggugccaugaugggcugcagcaacccccauccccacugccaggugugggccuccagcuuccuacccgacauugcacagcgagaggagcggagccaacaggcguacaagagccaacauggcgagccccugcucauggaguacucgaggcaagagcugcugcggaaggagaggcucguccugaccagcgagcacuggcuggugcuugugcccuucugggcaaccuggcccuaccagacccugcugcugccaaggaggcacgugcgcaggcucccggagcugacccccgccgagagagaugaccuggccuccaucaugaagaaacugcugacaaaguaugacaaccuguucgagacgucguuccccuacuccaugggguggcacggcgcccccacgggcagcgaggccggcgccaacuggaaucacuggcagcugcaugcccacuacuaucccccccugcugcguagcgcgaccgucaggaaauucauggucggcuacgagaugcuggcccaggcccagagggaccugacccccgagcaggccgccgagaggcugcgggcccugcccgagguccacuaucaccucggccagaaggaccgggaaaccgccacgaucgcg

SEQ ID NO: 17 - RNA, 1137 nt, Artificial Sequence
  GALT-CO13
auguccaggagcggcaccgacccccagcagaggcagcaggcuuccgaggccgacgccgccgccgccaccuucagggccaacgaccaccagcacauccguuacaacccgcugcaagacgaguggguccuaguguccgcccaccggaugaaacgccccuggcagggccagguggagccccaguugcugaagaccguacccaggcacgacccccugaacccgcucugccccggcgccaucagggccaacggcgaggugaacccccaauacgacagcaccuuccuguucgacaacgacuuccccgcccuccagccugaugcccccagcccgggccccagcgaccacccacuguuccaggccaaaagcgccaggggcgugugcaaggucaugugcuuccaccccuggucggacgugacgcugccccucauguccgugcccgagauccgcgccgugguggacgccugggccagcgugaccgaggagcugggcgcucaguaucccugggugcagaucuuugagaacaagggggccaugaugggcuguagcaacccccacccccacugccaggugugggccagcuccuuccugccagacaucgcccagcgugaggagcguucccagcaggccuacaaaagccagcacggugagccgcugcucauggaauacagccggcaggaacugcugcggaaggagcgucucgugcugacguccgagcacuggcuggugcugguuccguucugggccaccuggcccuaccagacccugcuccugcccaggcggcacgucagaaggcucccggagcugacccccgccgagcgggacgaccuggcgagcaucaugaagaagcugcugaccaaguacgacaaccuguucgagaccucauuccccuacagcaugggcuggcacggggcccccaccgggagcgaggccggcgcuaauuggaaccacuggcagcugcacgcccacuacuaccccccccugcugagguccgccaccguccgaaaguucaugguaggcuacgaaaugcuggcccaggcccaacgagaccugacccccgagcaagccgccgaacgcuugagggcccugcccgagguccacuaccaccugggccagaaggaccgggagacugccaccaucgcc

SEQ ID NO: 18 - RNA, 1137 nt, Artificial Sequence
  GALT-CO14
augagcagguccggcaccgacccucagcagaggcagcaggccagcgaggccgacgccgccgccgccacauuccgcgccaacgaucaccagcacauccgcuacaacccccugcaggacgagugggugcuggucagugcgcacaggaugaagaggccguggcagggccagguugagccccagcuccugaagacggugccacgucacgacccccucaacccccugugccccggcgcgauccgggcuaacggcgaggucaauccccaauacgacagcaccuuccuguucgacaacgacuuccccgcacugcagccggacgccccaagccccgggcccagcgaccacccccuguuucaagccaaaagcgccaggggcgucugcaaggugaugugcuuccaccccugguccgaugugacccugcccuugaugagcguccccgagauccgugccgugguggaugccugggccuccguuaccgaggagcugggcgcccaauacccaugggugcaaauauucgagaacaagggcgcgaugaugggcugcagcaacccccauccccauugucaggugugggccagcagcuuccucccggacaucgcccagcgcgaggaaaggagucagcaggccuacaagagccagcacggcgagccacugcugauggaguacagccgacaggagcugcugcggaaggagaggcuugugcucaccagcgagcacuggcuggugcugguccccuucugggccaccuggcccuaccaaacgcuccugcucccccggaggcaugugcgccgucugccagagcucacccccgccgagagggaugaccuggcgagcauuaugaagaagcugcugaccaaguaugauaaccuguuugagacgagcuuccccuacagcaugggauggcacggcgcccccaccggcuccgaggccggcgccaauuggaaccacuggcagcugcacgcccauuacuaccccccgcugcugcgguccgccaccgugaggaaauucauggugggguacgaaaugcuggcccaggcucagagggaccugacccccgagcaagcggccgagcggcugagggcgcugccugaggugcacuaccaucugggccaaaaggacagggaaaccgcaaccaucgcc

SEQ ID NO: 19 - RNA, 1137 nt, Artificial Sequence
  GALT-CO15
augagccgguccggaaccgacccccagcagaggcagcaggcaagcgaggccgacgccgccgcggccaccuuccgcgccaacgaucaccagcacauccgcuacaacccccugcaggacgagugggugcuggugagcgcccacaggaugaagcgccccuggcaggggcagguggagccgcagcugcugaagaccgugccccggcaugauccccugaacccccucugucccggcgccauaagggcgaauggcgaggucaacccccaguacgacagcacauuccuguucgacaacgacuuccccgcccugcagcccgacgcccccagccccggcccaagcgaucauccccucuuccaggccaagagcgcccggggggugugcaaagugaugugcuuccaccccugguccgacgugacccucccccucaugagcgugccugagauuagggccgugguggacgccugggccagcgugaccgaagagcugggagcccaguaccccugggugcagaucuucgaaaacaagggcgccaugaugggcuguuccaacccccauccccacugucaggugugggccagcagcuuucugcccgauaucgcccagagggaagagaggagccagcaggccuacaagucccagcacggagagccccugcugauggaguacagcaggcaagaacugcugaggaaggagcggcuggugcugaccagcgagcauuggcugguccuggugcccuucugggccaccuggccauaccagacccugcugcugccccgacggcacguccgcaggcugcccgagcugacccccgccgaaagggacgaccuggccagcaucaugaagaagcugcugacgaaguacgacaaccuguuugagaccagcuuccccuacagcaugggcuggcacggcgcccccacgggcagcgaggccggcgccaauuggaaucacuggcagcugcacgcccauuauuaccccccccuccugagguccgccaccgugcgaaaguuuauggucggcuacgagaugcuggcccaggcgcagcgagaucugacccccgagcaggccgccgagaggcugagggcccugcccgaagugcacuaccaccugggccagaaggacagggaaaccgccacgaucgcc

SEQ ID NO: 20 - RNA, 1137 nt, Artificial Sequence
  GALT-CO16
augagccggagcgggaccgauccccagcagaggcagcaggccagcgaagccgacgcagcagccgcaaccuuccgggccaacgaccaccagcauaucagguauaaucccuugcaagacgagugggugcucgucagcgcccaccggaugaagaggcccuggcaggggcaaguggagccccagcugcucaagaccgugccuaggcacgacccccucaacccgcugugcccuggcgccaucagggccaacggcgaggucaacccccaguaugacagcaccuuccuguucgacaacgacuuccccgcucuccagcccgacgccccaagccccggcccguccgaccacccccucuuccaggccaagucagcccggggcgucugcaaggugaugugcuuccaccccuggagcgacgucacgcugccccugaugagcgugcccgagauccgggccgugguggacgccugggccagcgugaccgaggagcugggcgcccaauaucccuggguccagaucuuugagaacaagggcgccaugaugggaugcagcaacccccacccccacugccaggucugggccagcagcuuccugcccgacaucgcccagagggaagagaggagccagcaagccuacaagucccagcacggcgagccucugcugauggaguacuccaggcaggagcugcucaggaaggagcggcuggugcucaccagcgaacacuggcuggugcuggugcccuuuugggccacauggcccuaccagacgcugcugcucccccgccgacaugugaggaggcugcccgagcugaccccagcggaaagggacgaccuggccagcaucaugaagaagcuccugaccaaguacgacaaccuguucgagaccagcuuccccuacagcaugggguggcauggcgcgcccaccggcagcgaggccggcgccaacuggaaucacuggcaacugcacgcccacuacuaccccccccugcuccggagugccaccgugaggaaguuuauggugggcuaugagaugcuggcccaggcccagcgugaccugaccccggaacaggcggccgagcgccugcgggcccugcccgaggugcacuaucaccucggccagaaggacagggagacagccaccaucgcc

SEQ ID NO: 21 - RNA, 1137 nt, Artificial Sequence
  GALT-CO17
augagccguuccggcaccgacccccagcagagacagcaggccagcgaggccgacgccgccgccgccacauuccgcgccaacgaccaccagcacaucagguacaauccccugcaagacgagugggugcuggugagcgcccaucggaugaagcggccauggcagggccagguggagccccagcuccugaagacggugcccaggcaugauccacugaacccccucugccccggcgccauccgggccaacggcgaggucaacccgcaguacgacagcaccuuccuguucgauaacgacuuccccgcccugcagcccgacgcccccuccccgggcccgagcgaucauccccuguuccaggccaagagcgccaggggggugugcaaagugaugugcuuccacccguggagcgacgucacccugccccugaugagcgugcccgagauccgugccgugguggacgccugggccagcgucacggaggagcucggggcccaguaccccugggugcagaucuucgaaaacaaaggcgcgaugauggggugcagcaacccacauccccacugccaggugugggccagcagcuuccuccccgacauagcccagagggaggagaggucucagcaggccuauaagucccagcacggggaaccccugcucauggaguacagccggcaggaacugcuccggaaggagaggcugguccugaccuccgagcacuggcucgugcucgugcccuucugggcgaccuggcccuaccagacccugcugcugccccggaggcacgugaggaggcugccggagcugaccccggccgagcgggacgaccuggccagcaucaugaagaagcugcugaccaaguacgauaaccuguucgagaccaguuuucccuacagcaugggguggcacggcgcccccaccggcagcgaggccggggccaacuggaaucauuggcagcugcacgcccacuauuaccccccccugcugaggucagccacggugaggaaguucauggugggguaugagaugcuggcccaggcccagcgggaccugacccccgagcaggccgccgagagacugagggcccuccccgaagugcacuaccaccuggggcagaaggaccgcgagaccgccaccauagcc

SEQ ID NO: 22 - RNA, 1137 nt, Artificial Sequence
  GALT-CO18
augagucggagcggcaccgacccccagcagaggcagcaggccagcgaggccgacgccgccgccgccaccuucagggccaacgaucaccagcacauccgcuacaacccccugcaggacgagugggugcuggugagcgcgcacaggaugaaaaggcccuggcagggccagguggagccccagcugcugaagaccgucccgaggcacgacccgcugaacccccugugccccggggcgaucagggcgaauggcgaggugaacccccaguacgacagcaccuuucuguuugacaaugauuucccagcccugcagcccgacgcccccucccccggccccagcgaccacccccuguuccaggccaagagcgccaggggcgugugcaaggucaugugcuuccaccccuggagcgacgugacccugcccuuaaugagcgugcccgaaaucagggccgugguggaugccugggcgagcgucacggaggaacugggcgcccaauaucccuggguacagaucuuugagaacaagggggccaugaugggcugcagcaauccccacccccacugccaagucugggcaagcagcuuccugcccgacaucgcgcagagggaggagcguagccagcaggcauacaagagccagcacggcgagccccugcugauggaguacagcaggcaggagcugcugagaaaggagcgucuggugcugaccagcgagcacuggcuggugcucguccccuucugggccaccuggcccuaccagacccuccugcugcccaggcggcacgugcgcaggcugcccgagcugacccccgccgaaagggacgacuuagccagcaucaugaagaaacuccugaccaaguaugacaaucuguucgagacguccuuccccuauuccaugggcuggcauggcgcaccgaccggaagcgaagccggggccaacuggaaccauuggcagcuccaugcgcacuacuaccccccccuccucagguccgccaccgugaggaaguucauggucggguacgagaugcuggcccaggcccagagggaccugacgcccgaacaggccgccgaacgccugagggcccugcccgagguacacuaccaccugggccagaaggacagggagaccgccaccaucgcc

SEQ ID NO: 23 - RNA, 1137 nt, Artificial Sequence
  GALT-CO19
augucccgcagcggcacggacccccagcagcggcagcaggcgagcgaggccgacgcugccgccgccaccuuucgcgcaaacgaccaucagcacaucagguauaacccacuccaggacgaguggguccugguguccgcccauaggaugaagcgacccuggcaggggcagguggagccccagcugcugaaaaccgugcccaggcacgacccccugaaucccuuaugccccggcgccauccgggccaacggcgaggugaacccacaguaugacuccaccuuucuguucgacaacgauuuccccgccuuacagcccgacgcccccagccccgguccgagcgaucacccccucuuccaggccaagagcgcgcgcggggugugcaaggugaugugcuuccaccccuggucggaugugacgcugccccucaugagcgugccggaaaucagggcggugguggacgcaugggccagcgugacagaggagcugggcgcccaauaccccugggugcagaucuucgagaacaagggcgcaaugaugggcugcagcaacccccacccccauugccaggugugggcgagcagcuuccugcccgacaucgcccagagggaggagaggucccagcaagccuauaaaucccagcauggugaaccccugcugauggaguacuccaggcaggagcugcugcggaaggagcgccugguccugaccuccgaacauuggcuggugcugguaccguucugggccaccuggcccuaccagacccugcugcucccccgccgacacgugcggaggcugccggagcugacccccgccgaacgggacgaccuggccuccauaaugaagaagcugcugaccaaguacgacaaccuguucgagaccuccuuccccuauagcaugggauggcacggggcccccaccggcagcgaggccggcgccaacuggaaccacuggcagcugcacgcccacuacuaccccccccugcugcgauccgccaccguccggaaguucauggugggcuacgagaugcuggcccaagcgcagcgggaccugacgcccgagcaggccgcggagcgucugcgcgcccuacccgaggugcacuaccaccugggccagaaagacagggagaccgccacaauagcc

SEQ ID NO: 24 - RNA, 1137 nt, Artificial Sequence
  GALT-CO20
augucccgcagcggcaccgacccccagcaacgacaacaagccagcgaggccgacgcggccgccgcaaccuuccgcgccaacgaccaucagcacauccgcuacaauccccuccaagacgagugggugcuggucagcgcccauaggaugaagcgcccguggcagggccagguggaaccgcagcuucugaagaccgugccgcgacacgacccccucaacccccugugccccggcgccaucagggcaaauggcgaggugaacccccaguacgacucgacguuucuguucgacaacgacuuucccgcccugcagcccgacgcccccucgcccggucccagcgaccacccccuguuccaggccaagagcgcccgcggcgugugcaaggugaugugcuuucaucccugguccgacgugacccugccccuuauguccgugccggagauccgcgccgugguggacgccugggccagcgucaccgaggagcugggggcccaguacccaugggugcagaucuucgaaaacaaaggugcaaugauggggugcagcaacccucacccccacugccaagucugggcgagcagcuuccucccggacauagcccagagggaggagcggucccagcaggccuacaagagccagcacggagagccccugcugauggaguacagccgccaggagcuccugcgcaaggagaggcugguccugaccagcgagcauuggcuggugcuggugcccuucugggccaccuggcccuaccagacccuccugcugccccggaggcacgugcggcggcugcccgaguugacccccgcggagcgcgaugaucuggccagcaucaugaagaaacugcugaccaaguacgacaaucuguuugagacauccuuccccuacagcaugggcuggcauggcgcccccacuggcagcgaggccggcgcgaacuggaaccauuggcagcugcacgcccacuacuacccaccccugcuccggagcgccacggugaggaaguucauggucggcuacgagaugcuggcccaggcccagagggaccugacgcccgagcaggccgcggaaaggcuucgcgcccugcccgaggugcacuaccaccuaggccaaaaggaucgggagaccgccaccaucgcc

SEQ ID NO: 25 - RNA, 1137 nt, Artificial Sequence
  GALT-CO21
augagcaggagcggcaccgacccccaacagagacagcaagccagcgaagccgacgccgcagccgcuaccuuccgggcuaacgaucaccagcacaucagguacaacccccuccaggacgagugggugcucguguccgcccauaggaugaagcgccccuggcaaggccagguggagccccagcugcugaagaccgugcccaggcacgacccccugaauccccugugccccggcgccauacgggccaacggggaggugaacccgcaguacgacagcaccuuccuguucgauaacgacuuccccgcccugcagccggacgccccaucccccggccccagcgaucacccccuguuccaggccaaguccgccaggggcgugugcaaggugauguguuuccaccccugguccgacgugacccugccccuuauguccgugccagagaucagggccguuguugacgccugggcguccgugaccgaggagcugggagcccaguaccccugggugcagaucuucgagaacaagggcgccaugaugggcuguagcaacccccacccgcauugccaagucugggccuccagcuuccugcccgacaucgcgcagcgagaggagcggagccaacaagccuacaagagccagcacggugagcccuugcugauggaguacagccggcaggagcuccugaggaaagagaggcucguucugaccuccgagcacuggcugguguuagugcccuucugggccaccuggcccuaccagacccugcugcugccccguaggcacgugcgccggcugcccgagcugacccccgccgagcgggaugaucuggccuccaucaugaaaaagcugcugaccaaguacgacaaucuguucgagaccagcuuccccuacagcaugggguggcacggcgcccccaccggcuccgaagccggcgccaacuggaaccacuggcagcuucacgcccacuauuauccgccccugcuccggagcgccaccguccgcaaauucauggugggcuacgagaugcuggcucaagcgcaacgcgaccugacccccgagcaggccgccgagaggcugagggcccugcccgaggugcacuaccaccugggccagaaagauagggagacggccaccaucgcc

SEQ ID NO: 26 - RNA, 1137 nt, Artificial Sequence
  GALT-CO22
auguccagguccggcaccgauccccaacagaggcagcaggccuccgaagccgacgccgccgccgccaccuucagggccaacgaccaucagcacauccgcuacaacccccugcaggacgagugggugcuggucagcgcccauaggaugaaacgcccguggcaggggcagguagagccacagcuccugaagaccgugccgaggcacgauccacucaacccccugugccccggcgccaucagggccaacggggaagugaacccccaguacgacuccaccuuucucuucgacaacgauuuccccgcccugcagccagacgccccgagccccggcccaagcgaucacccccuguuccaggccaagagcgcccguggcgugugcaaggugauguguuuccaccccuggagcgacgugacccugccccugaugagcgugcccgaaauccgcgcgguggucgaugccugggcaucagugaccgaggagcugggcgcccaauacccguggguacagaucuucgagaacaagggcgccaugaugggcuguagcaacccccauccccacugccaggugugggccagcucauuccuccccgacaucgcccagagggaggagaggucgcagcaggccuacaagucccagcacggggagccccuucugauggaguacagccggcaggaacugcugcggaaggaacggcuggugcugaccagcgagcacuggcuggugcuggugcccuuuugggccaccuggcccuaccagacccugcuacucccccggcggcacguccggcggcugcccgagcucacccccgccgagagagacgaccuggccuccaucaugaagaagcugcucaccaaauacgacaaucuguucgagaccagcuuccccuauagcaugggcuggcacggcgcgcccaccggcagcgaggccggggcgaacuggaaccauuggcaacuccacgcccacuacuaucccccccugcugaggagcgccacggugaggaaauucaugguagguuaugagaugcuggcccaggcccagagggaccugacccccgagcaggccgccgagaggcugagggcccugcccgaggugcauuaccaccuggggcagaaggacagggagaccgccaccauagcc

SEQ ID NO: 27 - RNA, 1137 nt, Artificial Sequence
  GALT-CO23
augucccggucaggcaccgacccacaacagcgccagcaggccagcgaggccgacgccgccgccgcgaccuucagggccaacgaccaccagcacaucagguacaacccccugcaggacgagugggugcuggugagcgcccacaggaugaagcgacccuggcagggucagguggagccccagcugcugaagaccguacccaggcacgacccccugaacccccucugcccgggggccaucagggccaacggagaggugaacccccaguacgacuccaccuuccuguuugauaacgacuuucccgcccugcagccugaugcccccagcccugggcccagcgaucacccccuguuccaggccaaaagcgccaggggagugugcaaagugaugugcuuccacccguggagcgaugugacccucccccugauguccguccccgagauccgagcagugguggacgccugggcgagcgugacggaggagcugggcgcgcaauaccccuggguccagaucuucgagaacaagggcgccaugauggggugcuccaacccccacccccacugccaggugugggcuuccuccuuccuccccgacaucgcccaaagggaggagaggagccagcaggccuacaagagccagcacggggagccucugcugauggaguacagcaggcaggaacugcugaggaaggagaggcuggugcuuaccuccgagcacuggcuggugcucguacccuucugggccaccuggcccuaccagacccugcugcugccccggaggcacgugcggaggcugcccgaacugacccccgcagagcgagacgaccucgccaguaucaugaagaaacugcugaccaaguaugacaaccuguucgagaccuccuuccccuacagcaugggcuggcacggcgcccccacgggcagcgaggccggugcuaacuggaaccacuggcagcugcacgcccacuacuaccccccccugcugaggagcgccaccgugaggaaguucauggugggguaugagaugcuggcccaggcccaacgugaccugacgcccgaacaggccgcagaacggcucagggcccugcccgaggugcacuaccaccugggccagaaggacagggagaccgccaccaucgcc

SEQ ID NO: 28 - RNA, 1137 nt, Artificial Sequence
  GALT-CO24
augagccgguccggcaccgacccccagcagcggcagcaggcauccgaggccgacgccgccgccgccaccuuccgggccaacgaccaucagcacauccguuauaacccacugcaagacgaguggguguuggugagcgcgcaucgcaugaaaaggccguggcaggggcagguggagccccagcugcugaagaccgucccccggcacgacccccugaacccucugugccccggcgccauccgggccaacggcgaggugaacccgcaauacgacagcacguuccuguucgauaacgacuuccccgcgcugcagcccgacgcccccagcccgggccccucggaccacccccuguuccaggccaagagcgcccguggcgucugcaaggucaugugcuuccaccccugguccgacgugacccucccccugaugagcgugcccgagauccgcgccgugguggacgccugggccuccgugaccgaggaacucggcgcgcaguaccccugggugcagauauucgagaacaaaggcgccaugaugggcugcuccaacccccacccccacugucaggucugggccucaagcuuccugcccgauaucgcccagcgcgaagagcggagccagcaggccuacaagagccagcacggggaaccccugcugauggaguacagccggcaggagcuccuacggaaggagaggcuggugcugaccuccgagcacuggcuggugcuggugcccuucugggcgaccuggcccuaucagacccugcuacugccccgcaggcacgugaggaggcugcccgaacugacccccgccgaaagggacgaccuggccuccauaaugaaaaagcugcugaccaaguacgacaaucuguucgagaccagcuuccccuacagcaugggcuggcacggugcccccaccggguccgaggccggcgccaauuggaaucacuggcagcugcaugcccauuauuaccccccccuccugcgaagcgccaccguccgcaaguucauggugggguacgaaaugcuggcccaggcacagcgggaccugacccccgagcaggccgccgagaggcugagggcgcugcccgaggugcacuaccaccuggggcaaaaggaccgggagaccgccacgaucgcc

SEQ ID NO: 29 - RNA, 1137 nt, Artificial Sequence
  GALT-CO25
augucccggagcggcaccgacccccaacagcggcagcaggcgagcgaagccgacgccgccgccgcaaccuuccgggccaacgaccaccagcacaucagguauaauccuuuacaggacgaguggguccuggugagcgcccacaggaugaagcggcccuggcaaggccagguggagccccagcugcugaagaccgugccgcgucacgaccccuugaacccucugugccccggcgccaucagggccaacggcgaggugaauccccaguacgacagcaccuuccuguucgacaacgacuuccccgcccugcagccagacgcccccucccccgggcccagcgaccauccccuguuccaggccaaaagcgcgcggggcgugugcaaggugaugugcuuucaccccuggagcgacgugacccugccgcugaugagcgugcccgagauccgcgccgucgucgacgcgugggccagcgugaccgaggagcugggcgcccaauacccgugggugcagaucuucgagaacaagggcgccaugauggggugcagcaacccgcacccccacugccaggugugggccagcagcuuccugcccgacaucgcgcaaagggaggagaggagccagcaggccuacaagagccagcacggugagccacugcugauggaauauagcaggcaggaacugcugaggaaagagaggcuggugcugaccuccgagcauuggcuggugcuggucccuuuuugggccaccuggcccuaccagacacuccugcuccccaggaggcacgugcgcaggcugcccgagcugaccccagccgagcgggacgaccucgccuccaucaugaaaaagcuccugaccaaguacgacaaccuguucgagaccuccuuuccguauagcaugggauggcacggcgcccccaccggcuccgaggccggcgccaacuggaaccacuggcaacugcaugcccauuacuacccaccccugcugcguuccgccaccgugcggaaguucaugguggguuacgagaugcucgcccaggcccagagggaucugacccccgagcaggccgccgagaggcugagggcccugcccgagguccacuaccaccuggggcaaaaggacagggagacugccaccauugcc

SEQ ID NO: 30 - RNA, 87 nt, Artificial Sequence
  miR-142
gacagugcagucacccauaaaguagaaagcacuacuaacagcacuggaggguguaguguuuccuacuuuauggaugaguguacugug

SEQ ID NO: 31 - RNA, 23 nt, Artificial Sequence
  miR-142-3p
uguaguguuuccuacuuuaugga

SEQ ID NO: 32 - RNA, 23 nt, Artificial Sequence
  miR-142-3p binding site
uccauaaaguaggaaacacuaca

SEQ ID NO: 33 - RNA, 21 nt, Artificial Sequence
  miR-142-5p
cauaaaguagaaagcacuacu

SEQ ID NO: 34 - RNA, 21 nt, Artificial Sequence
  miR-142-5p binding site
aguagugcuuucuacuuuaug

SEQ ID NO: 35 - RNA, 47 nt, Artificial Sequence
  5' UTR-001 (Upstream UTR)
gggaaauaagagagaaaagaagaguaagaagaaauauaagagccacc

SEQ ID NO: 36 - RNA, 47 nt, Artificial Sequence
  5' UTR-002 (Upstream UTR)
gggagaucagagagaaaagaagaguaagaagaaauauaagagccacc

SEQ ID NO: 37 - RNA, 145 nt, Artificial Sequence
  5' UTR-003
ggaauaaaagucucaacacaacauauacaaaacaaacgaaucucaagcaaucaagcauucuacuucuauugcagcaauuuaaaucauuucuuuuaaagcaaaagcaauuuucugaaaauuuucaccauuuacgaacgauagcaac

SEQ ID NO: 38 - RNA, 42 nt, Artificial Sequence
  5' UTR-004
gggagacaagcuuggcauuccgguacuguugguaaagccacc

SEQ ID NO: 39 - RNA, 47 nt, Artificial Sequence; identical to SEQ ID NO: 36
  5' UTR-005 (Upstream UTR)

SEQ ID NO: 40 - RNA, 145 nt, Artificial Sequence; identical to SEQ ID NO: 37
  5' UTR-006

SEQ ID NO: 41 - RNA, 42 nt, Artificial Sequence; identical to SEQ ID NO: 38
  5' UTR-007

SEQ ID NO: 42 - RNA, 47 nt, Artificial Sequence
  5' UTR-008
gggaauuaacagagaaaagaagaguaagaagaaauauaagagccacc

SEQ ID NO: 43 - RNA, 47 nt, Artificial Sequence
  5' UTR-009
gggaaauuagacagaaaagaagaguaagaagaaauauaagagccacc

SEQ ID NO: 44 - RNA, 47 nt, Artificial Sequence
  5' UTR-010
gggaaauaagagaguaaagaacaguaagaagaaauauaagagccacc

SEQ ID NO: 45 - RNA, 47 nt, Artificial Sequence
  5' UTR-011
gggaaaaaagagagaaaagaagacuaagaagaaauauaagagccacc

SEQ ID NO: 46 - RNA, 47 nt, Artificial Sequence
  5' UTR-012
gggaaauaagagagaaaagaagaguaagaagauauauaagagccacc

SEQ ID NO: 47 - RNA, 47 nt, Artificial Sequence
  5' UTR-013
gggaaauaagagacaaaacaagaguaagaagaaauauaagagccacc

SEQ ID NO: 48 - RNA, 47 nt, Artificial Sequence
  5' UTR-014
gggaaauuagagaguaaagaacaguaaguagaauuaaaagagccacc

SEQ ID NO: 49 - RNA, 47 nt, Artificial Sequence
  5' UTR-15 (Upstream UTR)
gggaaauaagagagaauagaagaguaagaagaaauauaagagccacc

SEQ ID NO: 50 - RNA, 47 nt, Artificial Sequence
  5' UTR-016 (Upstream UTR)
gggaaauaagagagaaaagaagaguaagaagaaaauuaagagccacc

SEQ ID NO: 51 - RNA, 47 nt, Artificial Sequence
  5' UTR-017 (Upstream UTR)
gggaaauaagagagaaaagaagaguaagaagaaauuuaagagccacc

SEQ ID NO: 52 - RNA, 92 nt, Artificial Sequence
  5' UTR-018 (Upstream UTR)
ucaagcuuuuggacccucguacagaagcuaauacgacucacuauagggaaauaagagagaaaagaagaguaagaagaaauauaagagccacc

SEQ ID NO: 53 - RNA, 142 nt, Artificial Sequence
  142-3p 3'UTR (UTR including miR142-3p binding site)
ugauaauaguccauaaaguaggaaacacuacagcuggagccucgguggccaugcuucuugccccuugggccuccccccagccccuccuccccuuccugcacccguacccccguggucuuugaauaaagucugagugggcggc

SEQ ID NO: 54 - RNA, 142 nt, Artificial Sequence
  142-3p 3'UTR (UTR including miR142-3p binding site)
ugauaauaggcuggagccucgguggcuccauaaaguaggaaacacuacacaugcuucuugccccuugggccuccccccagccccuccuccccuuccugcacccguacccccguggucuuugaauaaagucugagugggcggc

SEQ ID NO: 55 - RNA, 142 nt, Artificial Sequence
  142-3p 3'UTR (UTR including miR142-3p binding site)
ugauaauaggcuggagccucgguggccaugcuucuugccccuuccauaaaguaggaaacacuacaugggccuccccccagccccuccuccccuuccugcacccguacccccguggucuuugaauaaagucugagugggcggc

SEQ ID NO: 56 - RNA, 142 nt, Artificial Sequence
  142-3p 3'UTR (UTR including miR142-3p binding site)
ugauaauaggcuggagccucgguggccaugcuucuugccccuugggccuccccccaguccauaaaguaggaaacacuacaccccuccuccccuuccugcacccguacccccguggucuuugaauaaagucugagugggcggc

SEQ ID NO: 57 - RNA, 142 nt, Artificial Sequence
  142-3p 3'UTR (UTR including miR142-3p binding site)
ugauaauaggcuggagccucgguggccaugcuucuugccccuugggccuccccccagccccuccuccccuucuccauaaaguaggaaacacuacacugcacccguacccccguggucuuugaauaaagucugagugggcggc

SEQ ID NO: 58 - RNA, 142 nt, Artificial Sequence
  142-3p 3'UTR (UTR including miR142-3p binding site)
ugauaauaggcuggagccucgguggccaugcuucuugccccuugggccuccccccagccccuccuccccuuccugcacccguacccccuccauaaaguaggaaacacuacaguggucuuugaauaaagucugagugggcggc

SEQ ID NO: 59 - RNA, 142 nt, Artificial Sequence
  142-3p 3'UTR (UTR including miR142-3p binding site)
ugauaauaggcuggagccucgguggccaugcuucuugccccuugggccuccccccagccccuccuccccuuccugcacccguacccccguggucuuugaauaaaguuccauaaaguaggaaacacuacacugagugggcggc

SEQ ID NO: 60 - RNA, 371 nt, Artificial Sequence
  3' UTR-001
gcgccugcccaccugccaccgacugcuggaacccagccagugggagggccuggcccaccagaguccugcucccucacuccucgccccgcccccugucccagagucccaccugggggcucucuccacccuucucagaguuccaguuucaaccagaguuccaaccaaugggcuccauccucuggauucuggccaaugaaauaucucccuggcaggguccucuucuuuucccagagcuccaccccaaccaggagcucuaguuaauggagagcucccagcacacucggagcuugugcuuugucuccacgcaaagcgauaaauaaaagcauugguggccuuuggucuuugaauaaagccugaguaggaagucuaga

SEQ ID NO: 61 - RNA, 568 nt, Artificial Sequence
  3' UTR-002
gccccugccgcucccacccccacccaucugggccccggguucaagagagagcggggucugaucucguguagccauauagaguuugcuucugagugucugcuuuguuuaguagaggugggcaggaggagcugaggggcuggggcugggguguugaaguuggcuuugcaugcccagcgaugcgccucccugugggaugucaucacccugggaaccgggaguggcccuuggcucacuguguucugcaugguuuggaucugaauuaauuguccuuucuucuaaaucccaaccgaacuucuuccaaccuccaaacuggcuguaaccccaaauccaagccauuaacuacaccugacaguagcaauugucugauuaaucacuggccccuugaagacagcagaaugucccuuugcaaugaggaggagaucugggcugggcgggccagcuggggaagcauuugacuaucuggaacuugugugugccuccucagguauggcagugacucaccugguuuuaauaaaacaaccugcaacaucucauggucuuugaauaaagccugaguaggaagucuaga

SEQ ID NO: 62 - RNA, 289 nt, Artificial Sequence
  3' UTR-003 (alpha-actin UTR)
acacacuccaccuccagcacgcgacuucucaggacgacgaaucuucucaaugggggggcggcugagcuccagccaccccgcagucacuuucuuuguaacaacuuccguugcugccaucguaaacugacacaguguuuauaacguguacauacauuaacuuauuaccucauuuuguuauuuuucgaaacaaagcccuguggaagaaaauggaaaacuugaagaagcauuaaagucauucuguuaagcugcguaaauggucuuugaauaaagccugaguaggaagucuaga

SEQ ID NO: 63 - RNA, 379 nt, Artificial Sequence
  3' UTR-004 (Albumin UTR)
caucacauuuaaaagcaucucagccuaccaugagaauaagagaaagaaaaugaagaucaaaagcuuauucaucuguuuuucuuuuucguugguguaaagccaacacccugucuaaaaaacauaaauuucuuuaaucauuuugccucuuuucucugugcuucaauuaauaaaaaauggaaagaaucuaauagagugguacagcacuguuauuuuucaaagauguguugcuauccugaaaauucuguagguucuguggaaguuccaguguucucucuuauuccacuucgguagaggauuucuaguuucuugugggcuaauuaaauaaaucauuaauacucuucuaauggucuuugaauaaagccugaguaggaagucuaga

SEQ ID NO: 64 - RNA, 118 nt, Artificial Sequence
  3' UTR-005 (?-globin UTR
gcugccuucugcggggcuugccuucuggccaugcccuucuucucucccuugcaccuguaccucuuggucuuugaauaaagccugaguaggaaggcggccgcucgagcaugcaucuaga

SEQ ID NO: 65 - RNA, 908 nt, Artificial Sequence
  3' UTR-006 (G-CSF UTR)
gccaagcccuccccaucccauguauuuaucucuauuuaauauuuaugucuauuuaagccucauauuuaaagacagggaagagcagaacggagccccaggccucuguguccuucccugcauuucugaguuucauucuccugccuguagcagugagaaaaagcuccuguccucccauccccuggacugggagguagauagguaaauaccaaguauuuauuacuaugacugcuccccagcccuggcucugcaaugggcacugggaugagccgcugugagccccugguccugaggguccccaccugggacccuugagaguaucaggucucccacgugggagacaagaaaucccuguuuaauauuuaaacagcaguguuccccaucuggguccuugcaccccucacucuggccucagccgacugcacagcggccccugcauccccuuggcugugaggccccuggacaagcagagguggccagagcugggaggcauggcccuggggucccacgaauuugcuggggaaucucguuuuucuucuuaagacuuuugggacaugguuugacucccgaacaucaccgacgcgucuccuguuuuucuggguggccucgggacaccugcccugcccccacgagggucaggacugugacucuuuuuagggccaggcaggugccuggacauuugccuugcuggacggggacuggggaugugggagggagcagacaggaggaaucaugucaggccugugugugaaaggaagcuccacugucacccuccaccucuucaccccccacucaccaguguccccuccacugucacauuguaacugaacuucaggauaauaaaguguuugccuccauggucuuugaauaaagccugaguaggaaggcggccgcucgagcaugcaucuaga

SEQ ID NO: 66 - RNA, 835 nt, Artificial Sequence
  3' UTR-007 (Col1a2; collagen, type I, alpha 2 UTR)
acucaaucuaaauuaaaaaagaaagaaauuugaaaaaacuuucucuuugccauuucuucuucuucuuuuuuaacugaaagcugaauccuuccauuucuucugcacaucuacuugcuuaaauugugggcaaaagagaaaaagaaggauugaucagagcauugugcaauacaguuucauuaacuccuucccccgcucccccaaaaauuugaauuuuuuuuucaacacucuuacaccuguuauggaaaaugucaaccuuuguaagaaaaccaaaauaaaaauugaaaaauaaaaaccauaaacauuugcaccacuuguggcuuuugaauaucuuccacagagggaaguuuaaaacccaaacuuccaaagguuuaaacuaccucaaaacacuuucccaugagugugauccacauuguuaggugcugaccuagacagagaugaacugagguccuuguuuuguuuuguucauaauacaaaggugcuaauuaauaguauuucagauacuugaagaauguugauggugcuagaagaauuugagaagaaauacuccuguauugaguuguaucgugugguguauuuuuuaaaaaauuugauuuagcauucauauuuuccaucuuauucccaauuaaaaguaugcagauuauuugcccaaaucuucuucagauucagcauuuguucuuugccagucucauuuucaucuucuuccaugguuccacagaagcuuuguuucuugggcaagcagaaaaauuaaauuguaccuauuuuguauaugugagauguuuaaauaaauugugaaaaaaaugaaauaaagcauguuugguuuuccaaaagaacauau

SEQ ID NO: 67 - RNA, 297 nt, Artificial Sequence
  3' UTR-008 (Col6a2; collagen, type VI, alpha 2 UTR)
cgccgccgcccgggccccgcagucgagggucgugagcccaccccguccauggugcuaagcgggcccgggucccacacggccagcaccgcugcucacucggacgacgcccugggccugcaccucuccagcuccucccacgggguccccguagccccggcccccgcccagccccaggucuccccaggcccuccgcaggcugcccggccucccucccccugcagccaucccaaggcuccugaccuaccuggccccugagcucuggagcaagcccugacccaauaaaggcuuugaacccau

SEQ ID NO: 68 - RNA, 602 nt, Artificial Sequence
  3' UTR-009 (RPN1; ribophorin I UTR)
ggggcuagagcccucuccgcacagcguggagacggggcaaggagggggguuauuaggauuggugguuuuguuuugcuuuguuuaaagccgugggaaaauggcacaacuuuaccucugugggagaugcaacacugagagccaaggggugggaguugggauaauuuuuauauaaaagaaguuuuuccacuuugaauugcuaaaaguggcauuuuuccuaugugcagucacuccucucauuucuaaaauagggacguggccaggcacgguggcucaugccuguaaucccagcacuuugggaggccgaggcaggcggcucacgaggucaggagaucgagacuauccuggcuaacacgguaaaacccugucucuacuaaaaguacaaaaaauuagcugggcgugguggugggcaccuguagucccagcuacucgggaggcugaggcaggagaaaggcaugaauccaagaggcagagcuugcagugagcugagaucacgccauugcacuccagccugggcaacaguguuaagacucugucucaaauauaaauaaauaaauaaauaaauaaauaaauaaauaaaaauaaagcgagauguugcccucaaa

SEQ ID NO: 69 - RNA, 785 nt, Artificial Sequence
  3' UTR-010 (LRP1; low density lipoprotein receptor-related protein 1 UTR)
ggcccugccccgucggacugcccccagaaagccuccugcccccugccagugaaguccuucagugagccccuccccagccagcccuucccuggccccgccggauguauaaauguaaaaaugaaggaauuacauuuuauaugugagcgagcaagccggcaagcgagcacaguauuauuucuccauccccucccugccugcuccuuggcacccccaugcugccuucagggagacaggcagggagggcuuggggcugcaccuccuacccucccaccagaacgcaccccacugggagagcugguggugcagccuuccccucccuguauaagacacuuugccaaggcucuccccucucgccccaucccugcuugcccgcucccacagcuuccugagggcuaauucugggaagggagaguucuuugcugccccugucuggaagacguggcucugggugagguaggcgggaaaggauggaguguuuuaguucuugggggaggccaccccaaaccccagccccaacuccaggggcaccuaugagauggccaugcucaaccccccucccagacaggcccucccugucuccagggcccccaccgagguucccagggcuggagacuuccucugguaaacauuccuccagccuccccuccccuggggacgccaaggaggugggccacacccaggaagggaaagcgggcagccccguuuuggggacgugaacguuuuaauaauuuuugcugaauuccuuuacaacuaaauaacacagauauuguuauaaauaaaauugu

SEQ ID NO: 70 - RNA, 3001 nt, Artificial Sequence
  3' UTR-011 (Nnt1; cardiotrophin-like cytokine factor 1 UTR)
auauuaaggaucaagcuguuagcuaauaaugccaccucugcaguuuugggaacaggcaaauaaaguaucaguauacauggugauguacaucuguagcaaagcucuuggagaaaaugaagacugaagaaagcaaagcaaaaacuguauagagagauuuuucaaaagcaguaaucccucaauuuuaaaaaaggauugaaaauucuaaaugucuuucugugcauauuuuuuguguuaggaaucaaaaguauuuuauaaaaggagaaagaacagccucauuuuagauguaguccuguuggauuuuuuaugccuccucaguaaccagaaauguuuuaaaaaacuaaguguuuaggauuucaagacaacauuauacauggcucugaaauaucugacacaauguaaacauugcaggcaccugcauuuuauguuuuuuuuuucaacaaaugugacuaauuugaaacuuuuaugaacuucugagcuguccccuugcaauucaaccgcaguuugaauuaaucauaucaaaucaguuuuaauuuuuuaaauuguacuucagagucuauauuucaagggcacauuuucucacuacuauuuuaauacauuaaaggacuaaauaaucuuucagagaugcuggaaacaaaucauuugcuuuauauguuucauuagaauaccaaugaaacauacaacuugaaaauuaguaauaguauuuuugaagaucccauuucuaauuggagaucucuuuaauuucgaucaacuuauaauguguaguacuauauuaagugcacuugaguggaauucaacauuugacuaauaaaaugaguucaucauguuggcaagugauguggcaauuaucucuggugacaaaagaguaaaaucaaauauuucugccuguuacaaauaucaaggaagaccugcuacuaugaaauagaugacauuaaucugucuucacuguuuauaauacggauggauuuuuuuucaaaucaguguguguuuugaggucuuauguaauugaugacauuugagagaaaugguggcuuuuuuuagcuaccucuuuguucauuuaagcaccaguaaagaucaugucuuuuuauagaaguguagauuuucuuugugacuuugcuaucgugccuaaagcucuaaauauaggugaaugugugaugaauacucagauuauuugucucucuauauaauuaguuugguacuaaguuucucaaaaaauuauuaacacaugaaagacaaucucuaaaccagaaaaagaaguaguacaaauuuuguuacuguaaugcucgcguuuagugaguuuaaaacacacaguaucuuuugguuuuauaaucaguuucuauuuugcugugccugagauuaagaucuguguaugugugugugugugugugugcguuuguguguuaaagcagaaaagacuuuuuuaaaaguuuuaagugauaaaugcaauuuguuaauugaucuuagaucacuaguaaacucagggcugaauuauaccauguauauucuauuagaagaaaguaaacaccaucuuuauuccugcccuuuuucuucucucaaaguaguuguaguuauaucuagaaagaagcaauuuugauuucuugaaaagguaguuccugcacucaguuuaaacuaaaaauaaucauacuuggauuuuauuuauuuuugucauaguaaaaauuuuaauuuauauauauuuuuauuuaguauuaucuuauucuuugcuauuugccaauccuuugucaucaauuguguuaaaugaauugaaaauucaugcccuguucauuuuauuuuacuuuauugguuaggauauuuaaaggauuuuuguauauauaauuucuuaaauuaauauuccaaaagguuaguggacuuagauuauaaauuauggcaaaaaucuaaaaacaacaaaaaugauuuuuauacauucuauuucauuauuccucuuuuuccaauaagucauacaauugguagauaugacuuauuuuauuuuuguauuauucacuauaucuuuaugauauuuaaguauaaauaauuaaaaaaauuuauuguaccuuauagucugucaccaaaaaaaaaaaauuaucuguagguagugaaaugcuaauguugauuugucuuuaagggcuuguuaacuauccuuuauuuucucauuugucuuaaauuaggaguuuguguuuaaauuacucaucuaagcaaaaaauguauauaaaucccauuacuggguauauacccaaaggauuauaaaucaugcugcuauaaagacacaugcacacguauguuuauugcagcacuauucacaauagcaaagacuuggaaccaacccaaauguccaucaaugauagacuugauuaagaaaaugugcacauauacaccauggaauacuaugcagccauaaaaaaggaugaguucauguccuuuguagggacauggauaaagcuggaaaccaucauucugagcaaacuauugcaaggacagaaaaccaaacacugcauguucucacucauaggugggaauugaacaaugagaacacuuggacacaagguggggaacaccacacaccagggccugucaugggguggggggaguggggagggauagcauuaggagauauaccuaauguaaaugaugaguuaaugggugcagcacaccaacauggcacauguauacauauguagcaaaccugcacguugugcacauguacccuagaacuuaaaguauaauuaaaaaaaaaaagaaaacagaagcuauuuauaaagaaguuauuugcugaaauaaaugugaucuuucccauuaaaaaaauaaagaaauuuugggguaaaaaaacacaauauauuguauucuugaaaaauucuaagagaguggaugugaaguguucucaccacaaaagugauaacuaauugagguaaugcacauauuaauuagaaagauuuugucauuccacaauguauauauacuuaaaaauauguuauacacaauaaauacauacauuaaaaaauaaguaaaugua

SEQ ID NO: 71 - RNA, 1037 nt, Artificial Sequence
  3' UTR-012 (Col6a1; collagen, type VI, alpha 1 UTR)
cccacccugcacgccggcaccaaacccuguccucccaccccuccccacucaucacuaaacagaguaaaaugugaugcgaauuuucccgaccaaccugauucgcuagauuuuuuuuaaggaaaagcuuggaaagccaggacacaacgcugcugccugcuuugugcaggguccuccggggcucagcccugaguuggcaucaccugcgcagggcccucuggggcucagcccugagcuagugucaccugcacagggcccucugaggcucagcccugagcuggcgucaccugugcagggcccucuggggcucagcccugagcuggccucaccuggguuccccaccccgggcucuccugcccugcccuccugcccgcccucccuccugccugcgcagcuccuucccuaggcaccucugugcugcaucccaccagccugagcaagacgcccucucggggccugugccgcacuagccucccucuccucuguccccauagcugguuuuucccaccaauccucaccuaacaguuacuuuacaauuaaacucaaagcaagcucuucuccucagcuuggggcagccauuggccucugucucguuuugggaaaccaaggucaggaggccguugcagacauaaaucucggcgacucggccccgucuccugaggguccugcuggugaccggccuggaccuuggcccuacagcccuggaggccgcugcugaccagcacugaccccgaccucagagaguacucgcaggggcgcuggcugcacucaagacccucgagauuaacggugcuaaccccgucugcuccucccucccgcagagacuggggccuggacuggacaugagagccccuuggugccacagagggcugugucuuacuagaaacaacgcaaaccucuccuuccucagaauagugauguguucgacguuuuaucaaaggcccccuuucuauguucauguuaguuuugcuccuucuguguuuuuuucugaaccauauccauguugcugacuuuuccaaauaaagguuuucacuccucuc

SEQ ID NO: 72 - RNA, 577 nt, Artificial Sequence
  3' UTR-013 (Calr; calreticulin UTR)
agaggccugccuccagggcuggacugaggccugagcgcuccugccgcagagcuggccgcgccaaauaaugucucugugagacucgagaacuuucauuuuuuuccaggcugguucggauuugggguggauuuugguuuuguuccccuccuccacucucccccacccccuccccgcccuuuuuuuuuuuuuuuuuuaaacugguauuuuaucuuugauucuccuucagcccucaccccugguucucaucuuucuugaucaacaucuuuucuugccucuguccccuucucucaucucuuagcuccccuccaaccuggggggcagugguguggagaagccacaggccugagauuucaucugcucuccuuccuggagcccagaggagggcagcagaaggggguggugucuccaaccccccagcacugaggaagaacggggcucuucucauuucaccccucccuuucuccccugcccccaggacugggccacuucuggguggggcagugggucccagauuggcucacacugagaauguaagaacuacaaacaaaauuucuauuaaauuaaauuuugugucucc

SEQ ID NO: 73 - RNA, 2212 nt, Artificial Sequence
  3' UTR-014 (Col1a1; collagen, type I, alpha 1 UTR)
cucccuccaucccaaccuggcucccucccacccaaccaacuuuccccccaacccggaaacagacaagcaacccaaacugaacccccucaaaagccaaaaaaugggagacaauuucacauggacuuuggaaaauauuuuuuuccuuugcauucaucucucaaacuuaguuuuuaucuuugaccaaccgaacaugaccaaaaaccaaaagugcauucaaccuuaccaaaaaaaaaaaaaaaaaaagaauaaauaaauaacuuuuuaaaaaaggaagcuugguccacuugcuugaagacccaugcggggguaagucccuuucugcccguugggcuuaugaaaccccaaugcugcccuuucugcuccuuucuccacaccccccuuggggccuccccuccacuccuucccaaaucugucuccccagaagacacaggaaacaauguauugucugcccagcaaucaaaggcaaugcucaaacacccaaguggcccccacccucagcccgcuccugcccgcccagcacccccaggcccugggggaccugggguucucagacugccaaagaagccuugccaucuggcgcucccauggcucuugcaacaucuccccuucguuuuugagggggucaugccgggggagccaccagccccucacuggguucggaggagagucaggaagggccacgacaaagcagaaacaucggauuuggggaacgcgugucaaucccuugugccgcagggcugggcgggagagacuguucuguuccuuguguaacuguguugcugaaagacuaccucguucuugucuugaugugucaccggggcaacugccugggggcggggaugggggcaggguggaagcggcuccccauuuuauaccaaaggugcuacaucuaugugaugggugggguggggagggaaucacuggugcuauagaaauugagaugcccccccaggccagcaaauguuccuuuuuguucaaagucuauuuuuauuccuugauauuuuucuuuuuuuuuuuuuuuuuuuguggauggggacuugugaauuuuucuaaaggugcuauuuaacaugggaggagagcgugugcggcuccagcccagcccgcugcucacuuuccacccucucuccaccugccucuggcuucucaggccucugcucuccgaccucucuccucugaaacccuccuccacagcugcagcccauccucccggcucccuccuagucuguccugcguccucuguccccggguuucagagacaacuucccaaagcacaaagcaguuuuucccccuaggggugggaggaagcaaaagacucuguaccuauuuuguauguguauaauaauuugagauguuuuuaauuauuuugauugcuggaauaaagcauguggaaaugacccaaacauaauccgcaguggccuccuaauuuccuucuuuggaguugggggagggguagacauggggaaggggcuuuggggugaugggcuugccuuccauuccugcccuuucccuccccacuauucucuucuagaucccuccauaaccccacuccccuuucucucacccuucuuauaccgcaaaccuuucuacuuccucuuucauuuucuauucuugcaauuuccuugcaccuuuuccaaauccucuucuccccugcaauaccauacaggcaauccacgugcacaacacacacacacacucuucacaucugggguuguccaaaccucauacccacuccccuucaagcccauccacucuccacccccuggaugcccugcacuugguggcggugggaugcucauggauacugggagggugaggggaguggaacccgugaggaggaccugggggccucuccuugaacugacaugaagggucaucuggccucugcucccuucucacccacgcugaccuccugccgaaggagcaacgcaacaggagaggggucugcugagccuggcgagggucugggagggaccaggaggaaggcgugcucccugcucgcuguccuggcccugggggagugagggagacagacaccugggagagcuguggggaaggcacucgcaccgugcucuugggaaggaaggagaccuggcccugcucaccacggacugggugccucgaccuccugaauccccagaacacaaccccccugggcugggguggucuggggaaccaucgugcccccgccucccgccuacuccuuuuuaagcuu

SEQ ID NO: 74 - RNA, 729 nt, Artificial Sequence
  3' UTR-015 (Plod1; procollagen-lysine, 2-oxoglutarate 5-dioxygenase 1 UTR)
uuggccaggccugacccucuuggaccuuucuucuuugccgacaaccacugcccagcagccucugggaccucggggucccagggaacccaguccagccuccuggcuguugacuucccauugcucuuggagccaccaaucaaagagauucaaagagauuccugcaggccagaggcggaacacaccuuuauggcuggggcucuccgugguguucuggacccagccccuggagacaccauucacuuuuacugcuuuguagugacucgugcucuccaaccugucuuccugaaaaaccaaggcccccuucccccaccucuuccauggggugagacuugagcagaacaggggcuuccccaaguugcccagaaagacugucugggugagaagccauggccagagcuucucccaggcacagguguugcaccagggacuucugcuucaaguuuugggguaaagacaccuggaucagacuccaagggcugcccugagucugggacuucugccuccauggcuggucaugagagcaaaccguaguccccuggagacagcgacuccagagaaccucuugggagacagaagaggcaucugugcacagcucgaucuucuacuugccuguggggaggggagugacagguccacacaccacacugggucacccuguccuggaugccucugaagagagggacagaccgucagaaacuggagaguuucuauuaaaggucauuuaaacca

SEQ ID NO: 75 - RNA, 847 nt, Artificial Sequence
  3' UTR-016 (Nucb1; nucleobindin 1 UTR)
uccuccgggaccccagcccucaggauuccugaugcuccaaggcgacugaugggcgcuggaugaaguggcacagucagcuucccugggggcuggugucauguugggcuccuggggcgggggcacggccuggcauuucacgcauugcugccaccccagguccaccugucuccacuuucacagccuccaagucuguggcucuucccuucuguccuccgaggggcuugccuucucucguguccagugaggugcucagugaucggcuuaacuuagagaagcccgcccccuccccuucuccgucugucccaagagggucugcucugagccugcguuccuagguggcucggccucagcugccuggguuguggccgcccuagcauccuguaugcccacagcuacuggaauccccgcugcugcuccgggccaagcuucugguugauuaaugagggcaugggguggucccucaagaccuuccccuaccuuuuguggaaccagugaugccucaaagacaguguccccuccacagcugggugccaggggcaggggauccucaguauagccggugaacccugauaccaggagccugggccucccugaaccccuggcuuccagccaucucaucgccagccuccuccuggaccucuuggcccccagccccuuccccacacagccccagaagggucccagagcugaccccacuccaggaccuaggcccagccccucagccucaucuggagccccugaagaccagucccacccaccuuucuggccucaucugacacugcuccgcauccugcuguguguccuguuccauguuccgguuccauccaaauacacuuucuggaacaaa

SEQ ID NO: 76 - RNA, 110 nt, Artificial Sequence
  3' UTR-017 (?-globin)
gcuggagccucgguggccaugcuucuugccccuugggccuccccccagccccuccuccccuuccugcacccguacccccguggucuuugaauaaagucugagugggcggc

SEQ ID NO: 77 - RNA, 119 nt, Artificial Sequence
  3' UTR-018
ugauaauaggcuggagccucgguggccaugcuucuugccccuugggccuccccccagccccuccuccccuuccugcacccguacccccguggucuuugaauaaagucugagugggcggc

SEQ ID NO: 78 - DNA, 18 bp, Artificial Sequence
  Syn'5 Promoter
attgggcacccgtaaggg

SEQ ID NO: 79 - RNA, 133 nt, Artificial Sequence
  (3' UTR with miR 142-3p binding site)
gcuggagccucgguggccaugcuucuugccccuugggccuccccccagccccuccuccccuuccugcacccguacccccuccauaaaguaggaaacacuacaguggucuuugaauaaagucugagugggcggc

SEQ ID NO: 80 - RNA, 22 nt, Artificial Sequence
  (miR 146-3p sequence)
ccucugaaauucaguucuucag

SEQ ID NO: 81 - RNA, 22 nt, Artificial Sequence
  (miR 146-5p sequence)
ugagaacugaauuccauggguu

SEQ ID NO: 82 - RNA, 22 nt, Artificial Sequence
  (miR 155-3p sequence)
cuccuacauauuagcauuaaca

SEQ ID NO: 83 - RNA, 23 nt, Artificial Sequence
  (miR 155-5p sequence)
uuaaugcuaaucgugauaggggu

SEQ ID NO: 84 - RNA, 22 nt, Artificial Sequence
  (miR 126-3p sequence)
ucguaccgugaguaauaaugcg

SEQ ID NO: 85 - RNA, 21 nt, Artificial Sequence
  miR-126-5p
cauuauuacuuuugguacgcg

SEQ ID NO: 86 - RNA, 22 nt, Artificial Sequence
  miR 16-3p sequence
ccaguauuaacugugcugcuga

SEQ ID NO: 87 - RNA, 22 nt, Artificial Sequence
  (miR 16-5p sequence)
uagcagcacguaaauauuggcg

SEQ ID NO: 88 - RNA, 21 nt, Artificial Sequence
  miR 21-3p sequence
caacaccagucgaugggcugu

SEQ ID NO: 89 - RNA, 22 nt, Artificial Sequence
  (miR 21-5p sequence)
uagcuuaucagacugauguuga

SEQ ID NO: 90 - RNA, 22 nt, Artificial Sequence
  (miR 223-3p sequence)
ugucaguuugucaaauacccca

SEQ ID NO: 91 - RNA, 22 nt, Artificial Sequence
  (miR 223-5p sequence)
cguguauuugacaagcugaguu

SEQ ID NO: 92 - RNA, 22 nt, Artificial Sequence
  (miR 24-3p sequence)
uggcucaguucagcaggaacag

SEQ ID NO: 93 - RNA, 22 nt, Artificial Sequence
  (miR 24-5p sequence)
ugccuacugagcugauaucagu

SEQ ID NO: 94 - RNA, 21 nt, Artificial Sequence
  (miR 27-3p sequence)
uucacaguggcuaaguuccgc

SEQ ID NO: 95 - RNA, 22 nt, Artificial Sequence
  (miR 27-5p sequence)
agggcuuagcugcuugugagca

SEQ ID NO: 96 - RNA, 22 nt, Artificial Sequence
  (miR 126-3p binding site)
cgcauuauuacucacgguacga

SEQ ID NO: 97 - RNA, 141 nt, Artificial Sequence
  (3' UTR with miR 126-3p binding site)
ugauaauaggcuggagccucgguggccaugcuucuugccccuugggccuccccccagccccuccuccccuuccugcacccguaccccccgcauuauuacucacgguacgaguggucuuugaauaaagucugagugggcggc

SEQ ID NO: 98 - RNA, 164 nt, Artificial Sequence
  3' UTR (miR142+miR126 binding sites variant 1)
ugauaauaguccauaaaguaggaaacacuacagcuggagccucgguggccaugcuucuugccccuugggccuccccccagccccuccuccccuuccugcacccguaccccccgcauuauuacucacgguacgaguggucuuugaauaaagucugagugggcggc

SEQ ID NO: 99 - RNA, 23 nt, Artificial Sequence
  miR 155-5p sequence)
uuaaugcuaauugugauaggggu

SEQ ID NO: 100 - RNA, 23 nt, Artificial Sequence
  (miR 155-5p binding site)
accccuaucacaauuagcauuaa

SEQ ID NO: 101 - RNA, 188 nt, Artificial Sequence
  (3 UTR with 3 miR 142-3p binding sites)
ugauaauaguccauaaaguaggaaacacuacagcuggagccucgguggccaugcuucuugccccuugggccuccauaaaguaggaaacacuacauccccccagccccuccuccccuuccugcacccguacccccuccauaaaguaggaaacacuacaguggucuuugaauaaagucugagugggcggc

SEQ ID NO: 102 - RNA, 140 nt, Artificial Sequence
  3' UTR with miR 142-5p binding site)
ugauaauaggcuggagccucgguggccaugcuucuugccccuugggccuccccccagccccuccuccccuuccugcacccguacccccaguagugcuuucuacuuuaugguggucuuugaauaaagucugagugggcggc

SEQ ID NO: 103 - RNA, 182 nt, Artificial Sequence
  (3' UTR with 3 miR 142-5p binding sites)
ugauaauagaguagugcuuucuacuuuauggcuggagccucgguggccaugcuucuugccccuugggccaguagugcuuucuacuuuauguccccccagccccuccuccccuuccugcacccguacccccaguagugcuuucuacuuuaugguggucuuugaauaaagucugagugggcggc

SEQ ID NO: 104 - RNA, 184 nt, Artificial Sequence
  (3' UTR with 2 miR 142-5p binding sites and 1 miR 142-3p binding site)
ugauaauagaguagugcuuucuacuuuauggcuggagccucgguggccaugcuucuugccccuugggccuccauaaaguaggaaacacuacauccccccagccccuccuccccuuccugcacccguacccccaguagugcuuucuacuuuaugguggucuuugaauaaagucugagugggcggc

SEQ ID NO: 105 - RNA, 142 nt, Artificial Sequence
  (3' UTR with miR 155-5p binding site)
ugauaauaggcuggagccucgguggccaugcuucuugccccuugggccuccccccagccccuccuccccuuccugcacccguacccccaccccuaucacaauuagcauuaaguggucuuugaauaaagucugagugggcggc

SEQ ID NO: 106 - RNA, 188 nt, Artificial Sequence
  (3' UTR with 3 miR 155-5p binding sites)
ugauaauagaccccuaucacaauuagcauuaagcuggagccucgguggccaugcuucuugccccuugggccaccccuaucacaauuagcauuaauccccccagccccuccuccccuuccugcacccguacccccaccccuaucacaauuagcauuaaguggucuuugaauaaagucugagugggcggc

SEQ ID NO: 107 - RNA, 188 nt, Artificial Sequence
  (3' UTR with 2 miR 155-5p binding sites and 1 miR 142-3p binding site)
ugauaauagaccccuaucacaauuagcauuaagcuggagccucgguggccaugcuucuugccccuugggccuccauaaaguaggaaacacuacauccccccagccccuccuccccuuccugcacccguacccccaccccuaucacaauuagcauuaaguggucuuugaauaaagucugagugggcggc

SEQ ID NO: 108 - RNA, 142 nt, Artificial Sequence
  (3' UTR with miR 142-3p binding site, P3 insertion)
ugauaauaggcuggagccucgguggccaugcuucuugccccuugggccuccauaaaguaggaaacacuacauccccccagccccuccuccccuuccugcacccguacccccguggucuuugaauaaagucugagugggcggc

SEQ ID NO: 109 - RNA, 70 nt, Artificial Sequence
  (5' UTR with miR142-3p binding site at position p1)
gggaaauaagaguccauaaaguaggaaacacuacaagaaaagaagaguaagaagaaauauaagagccacc

SEQ ID NO: 110 - RNA, 70 nt, Artificial Sequence
  (5' UTR with miR142-3p binding site at position p2)
gggaaauaagagagaaaagaagaguaauccauaaaguaggaaacacuacagaagaaauauaagagccacc

SEQ ID NO: 111 - RNA, 70 nt, Artificial Sequence
  (5' UTR with miR142-3p binding site at position p3)
gggaaauaagagagaaaagaagaguaagaagaaauauaauccauaaaguaggaaacacuacagagccacc

SEQ ID NO: 112 - RNA, 181 nt, Artificial Sequence
  (3' UTR with 3 miR 142-5p binding sites)
ugauaauagaguagugcuuucuacuuuauggcuggagccucgguggccaugcuucuugccccuugggccaguagugcuuucuacuuuauguccccccagccccucuccccuuccugcacccguacccccaguagugcuuucuacuuuaugguggucuuugaauaaagucugagugggcggc

SEQ ID NO: 113 - RNA, 1137 nt, Artificial Sequence
  GALT-CO26
augucuaggagcgggaccgacccccagcagcggcagcaggccagcgaggccgacgccgccgcggccaccuucagggccaacgaccaucaacacaucagguauaacccccuccaggacgaguggguguugguguccgcccaucggaugaagaggcccuggcagggccagguggagccccagcuccugaagaccgugccccggcacgacccccucaacccccugugccccggcgcgauccgcgccaacggcgaggugaacccccaguaugacagcacguuccuguucgacaacgacuuccccgcccugcagcccgacgcccccagccccggcccaagcgaccauccccuguuccaggccaaguccgccaggggcguguguaaggugaugugcuuccacccaugguccgacgugacccugccccugaugagcgugcccgagauccgcgccgugguggacgccugggccagcgugaccgaggagcugggggcccaguacccuugggugcaaaucuucgagaauaagggcgccaugaugggcugcuccaacccccacccccacugucaggugugggccagcaguuuccugcccgacaucgcccagcgcgaggagcggucacagcaggccuacaagagccaacacggcgaaccucugcucauggaguacagcaggcaggaacugcugcggaaggagaggcugguccugaccagcgagcacuggcuggugcuggugcccuucugggccaccuggcccuaccagacacugcugcugccuaggcgacacgugcgucggcugcccgagcugaccccugccgaaagggacgaccuggccagcaucaugaagaagcugcucaccaaguacgacaaccuguuugaaaccagcuuccccuacagcaugggcuggcacggcgcaccuaccggcagcgaggccggcgccaacuggaaccacuggcagcugcaugcccacuacuauccgccccuccucaggagcgccaccgugcgcaaguucauggugggcuaugagaugcuggcgcaggcccagcgugaccugacccccgagcaggccgccgagaggcugcgugcccugccugaggugcacuaccaccuggggcagaaggacagagaaacugcgaccaucgcc

SEQ ID NO: 114 - RNA, 1137 nt, Artificial Sequence
  GALT-CO27
augagcagguccggcaccgacccccagcagaggcagcaagccuccgaggccgacgccgccgcggccaccuuccgggccaacgaccaucagcauaucagguauaacccccuucaggacgagugggugcucgugagcgcccaccggaugaagcgccccuggcaggggcaggucgagccccagcugcugaagaccgugcccaggcacgauccgcugaacccgcugugccccggggccauccgggccaacggggaggugaacccccaguacgacagcaccuuccuguucgacaacgacuuccccgcccugcagcccgaugcccccagccccgggcccuccgaccacccccuguuccaggccaagagcgccagaggcgugugcaaggucaugugcuuucaucccuggagcgacgugacccugccccugauguccgugcccgagaucagagcugucguggacgccugggccuccgugaccgaggagcucggcgcccaguaccccugggugcagaucuucgagaacaaaggcgccaugaugggcugcagcaacccccacccacacugccaggugugggccagcagcuuccugcccgacaucgcccagagagaggagaggagccagcaggccuauaagagccagcauggcgagccccugcugauggaguacagcagacaggagcugcugaggaaagagaggcuggugcugacaagcgagcacuggcuggugcuggugcccuuuugggccacuuggccauaccagacccugcugcugccccggcggcaugucaggagacugccugagcugacucccgccgagcgggaugaccuggccagcaucaugaagaagcugcucaccaaauacgacaaccucuucgaaaccagcuuccccuacagcaugggguggcacggggcccccaccggcagcgaagccggagccaauuggaaucauuggcagcuccaugcccauuacuauccgccccugcucagaagcgccaccgugcggaaguucauggugggcuacgagaugcucgcccaggcccagcgggaccugacccccgagcaggcugccgagcggcugagggcccugcccgaggugcacuaucaccugggccagaaagauagggaaacagccacuaucgcc

SEQ ID NO: 115 - RNA, 1137 nt, Artificial Sequence
  GALT-CO28
augagcaggagcggcaccgacccccagcagaggcagcaggccagcgaagccgacgccgccgccgccaccuuccgggccaacgaucaccagcacauccgcuacaacccucuccaggacgagugggugcucgugagcgcccacaggaugaagcggcccuggcagggccagguggagccccagcuccugaagaccgugcccagacacgacccccugaacccgcucugccccggcgccaucagagccaacggcgaggugaacccccaguacgacagcaccuuccuguucgacaacgacuuccccgcccuccagcccgaugcccccagccccggucccuccgaccauccccuguuccaggccaaguccgccagaggcgugugcaaggugaugugcuuccaccccuggagcgacgugacccucccccugaugucggugcccgaaaucagggccgugguggacgccugggccagcgugaccgaggagcugggggcccaguaucccuggguccagaucuucgagaacaagggggccaugaugggcuguagcaacccccacccacacugccaggugugggccuccuccuuccugcccgacaucgcccaaagggaggagcggucccagcaagccuacaagucccagcacggugagccccugcugauggaauauagcagacaggagcugcugaggaaggagcgccugguccugaccagcgagcacuggcuggugcugguccccuuuugggccaccuggcccuaccagacgcugcugcugccucgcagacaugugaggaggcugccggagcugacccccgccgagcgggacgaccuggcaagcaucaugaagaagcugcugaccaaguacgacaaccuguucgagacuuccuucccguacagcaugggcuggcacggcgccccgaccggaagcgaggccggcgcgaacuggaaccacuggcagcugcaugcgcauuacuacccgccccugcugcggucagccaccguccgcaaguucauggugggcuacgaaaugcuggcccaggcgcagagggaccucacccccgagcaggccgccgaaagacugcgugcgcugccggaggugcacuaccaccugggccagaaggaccgcgaaaccgcgaccaucgca

SEQ ID NO: 116 - RNA, 1137 nt, Artificial Sequence
  GALT-CO29
augucacggagcggcaccgacccgcagcagaggcagcaggccagcgaggcagacgccgccgccgccaccuucagggccaacgaccaucagcacaucagauacaacccccuacaggacgagugggugcucgucagcgcccacagaaugaagcggcccuggcaggggcagguggagccccagcuccugaagaccgugcccaggcacgacccccucaauccccugugcccuggcgccauuagggccaacggcgaggugaacccccaguacgacucaaccuuccuguuugacaacgacuuccccgcccugcagcccgaugccccgagccccgggcccagcgaccacccccuguuccaggccaagucggccaggggcgugugcaaggugaugugcuuccaccccuggagcgaugucacccugccccugaugucggugcccgagauccgcgccgugguggacgccugggccagcgugaccgaggagcugggcgcccaauaccccugggugcagaucuuugagaacaaaggcgccaugaugggcuguagcaacccccacccccacugucaggugugggccagcagcuuucugcccgacaucgcccagagggaggagcgcucccagcaggcuuacaagagccagcacggagagccccugcucauggaguacucgcgacaggagcugcuccggaaggaacggcugguccugaccuccgagcacuggcucgugcuggugccguucugggccacauggcccuaccagacccugcugcuaccccgcagacacguucgccgacugcccgagcugaccccugccgagagagacgaccuggcgagcaucaugaagaagcugcucaccaaguaugacaacuuauucgaaaccuccuucccuuacagcaugggcuggcacggcgcccccaccggcagcgaggcgggcgccaacuggaaccacuggcagcugcaugcccacuacuacccaccccugcugcggagcgccaccgugagaaaguucauggugggcuacgagaugcuggcccaggcccaacgggaucugacccccgagcaggccgccgagcggcugagggcccuccccgagguacacuaccaucucggccagaaggaccgggaaaccgccaccaucgcc

SEQ ID NO: 117 - RNA, 1137 nt, Artificial Sequence
  GALT-CO30
augagcagaagcggcaccgacccccagcagcggcagcaggccagcgaggccgacgccgccgccgcaaccuuccgcgccaacgaccaccagcacaucagauacaacccccuccaggacgaguggguccucguguccgcccauagaaugaagaggccauggcagggccagguagaaccucaacugcugaagaccgucccccggcaugacccccucaauccccucugcccgggggccauccgagcgaauggggaggucaacccccaguacgacagcaccuuccuguucgacaacgacuuccccgcccugcagcccgacgccccgagccccggacccagcgaccacccccuguuccaggccaaauccgcccggggcgucugcaaggugaugugcuuucaccccugguccgacgugacccugccccucauguccgugcccgagaucagggccgugguggacgcuugggccagcgucacggaggagcucggcgcccaguaccccuggguccagaucuucgagaacaagggcgccaugauggggugcuccaacccucacccccacugccaggugugggccagcagcuuucugcccgacauugcccagcgggaggagaggucccagcaggccuacaagagucagcacggggagccccugcugauggaguacucccggcaggagcuccugaggaaagagcgcuuggugcugacaagcgagcacuggcuggugcucgugcccuucugggccacuuggcccuaccagacccugcugcugcccagacggcacgugcggcggcugcccgagcugacacccgccgagagggacgaucucgccagcauuaugaagaagcugcugaccaaguaugacaaccuguuugagacuagcuuucccuacagcaugggcuggcacggggcccccacgggcuccgaggccggcgccaacuggaaccacuggcagcugcacgcccacuauuauccgccccugcuccggagcgccaccgugagaaaguuuauggugggcuaugagaugcuggcccaagcgcaacgggaucugacccccgagcaggccgccgagcgucugagagcccugccugaggugcacuaucaccuggggcagaaggaccgggagacggcaaccaucgcc

SEQ ID NO: 118 - RNA, 1137 nt, Artificial Sequence
  GALT-CO31
augagccgcagcggcaccgacccgcaacaaagacagcaggccuccgaggccgacgccgccgccgcuaccuuuagggccaacgaccaccagcauauccgcuacaauccccuccaggacgagugggugcucgugagcgcccaccguaugaagaggcccuggcagggacagguggaaccccagcugcugaagaccguaccccggcacgacccccugaacccccugugccccggggccaucagagccaauggagaggugaacccccaguacgacuccaccuuccuguucgauaaugauuuuccggcccugcagcccgacgcccccagccccggcccaagcgaccacccucuguuccaggccaagagcgccaggggcguuugcaaggucaugugcuuccaccccuggagcgacgugacccugccccugaugucggugcccgagaucagggccgugguggacgccugggccagcgugacggaggaacucggcgcccaguaccccuggguacagaucuucgagaacaagggugccaugaugggcugcagcaacccacauccccacugucaggugugggccagcucauuccugccugacaucgcccagcgugaggagaggagucagcaggccuauaagagccagcauggggagccccuccugauggaguacagcagacaagagcugcucaggaaggagagacuggugcugaccagcgagcauuggcuggugcuggugcccuuuugggccacauggcccuaccagacccuccugcugccgagacgccacgugcgccggcugcccgagcugacucccgccgagagggacgaccucgcuagcaucaugaagaaacugcugaccaaguacgacaaccuguuugagacaagcuuucccuacuccaugggauggcacggcgcccccaccggcuccgaggccggcgccaacuggaaccacuggcagcugcacgcccacuacuaucccccgcugcugcggagcgccaccgugaggaaauucauggugggcuacgagaugcucgcucaggcccaacgggaccugacccccgagcaggcggccgagaggcuccgagcucugcccgaggugcauuaccaucugggccagaaggauagggaaaccgccaccaucgcc

SEQ ID NO: 119 - RNA, 1137 nt, Artificial Sequence
  GALT-CO32
augagcaggagcggaaccgacccgcagcagaggcagcaggccagcgaagccgacgccgccgccgccaccuuccgggccaacgaccaccaacacaucagguacaacccgcuccaggacgagugggugcucguuagcgcccaucgcaugaagcggccguggcaaggccagguggagccgcagcugcugaagaccgugccgcgccacgacccgcugaacccgcugugcccuggcgccauccgggccaacggcgaggugaacccucaguacgacagcaccuuccuguucgacaaugauuucccggccuugcagccggacgccccuuccccgggaccguccgaccacccgcuguuccaagccaaguccgcccggggcgugugcaaggugaugugcuuccacccgugguccgacgugacccugccgcugaugagcgugccugagaucagagccgugguggacgccugggccuccgugacugaggagcucggcgcccaguacccauggguccagaucuucgagaacaagggugccaugaugggcugcagcaacccgcacccgcacugccaagugugggccagcuccuuccugccggauauugcccagcgggaggagcggagccagcaagcauacaagagccagcauggcgagccgcucuugauggaguacuccaggcaggagcugcugagaaaggagcggcuggugcugaccucugagcacuggcuggugcucgugccguucugggccaccuggccuuaccagacccugcugcugccgaggcggcacgugcgccggcugccagagcugacgccagccgagcgagacgaucuggccuccaucaugaagaagcuacugaccaaguaugacaaccuguucgaaacgagcuucccguacagcaugggcuggcacggcgccccgaccggcagcgaggccggcgccaacuggaaucacuggcagcugcaugcccauuacuacccgccgcuccuccgcagcgccaccgugaggaaguucauggugggcuacgagaugcuggcccaggcccagcgggaccugaccccggagcaggcggccgagagacugagggcccucccggagguccauuaccaccugggccagaaggaccgggagacggccaccaucgcc

SEQ ID NO: 120 - RNA, 1137 nt, Artificial Sequence
  GALT-CO33
augucccgcagcggcacggacccgcagcagcggcagcaggccagcgaggccgacgccgcggccgccaccuuccgggccaacgaccaccagcacaucagguacaacccacuccaagacgagugggugcucgugagcgcccaccggaugaagaggccguggcagggacagguugagccgcaacugcugaagaccgugccaagacacgauccgcugaacccgcucugcccgggcgccauccgugccaacggcgaggucaacccacaguaugacagcaccuuccuguucgacaacgacuucccggcccugcagccggacgcgccuagcccuggaccguccgaccacccgcuguuccaggccaaguccgcuaggggcgugugcaaggugaugugcuuccauccgugguccgaugucacccugccgcucauguccgugccggagauccgggccgugguggaugccugggccagcgucaccgaggagcugggcgcgcaguacccuuggguccagaucuucgagaacaagggcgccaugauggguugcagcaacccgcacccacacugccaggugugggccagcagcuuccugccggacaucgcacagagggaggagcggagccaacaggccuacaagucccagcacggcgagccacugcugauggaguacagcaggcaggagcugcugcggaaggagcggcuggugcucaccuccgaacauuggcugguucuggugccguucugggccaccuggccuuaccagacccugcugcucccgaggcggcacgugcgcaggcugccggagcugacaccggccgagcgcgacgaccuggccagcaucaugaagaagcugcucaccaaguacgauaaccuguucgagacauccuucccguacagcaugggcuggcacggcgccccuaccggcuccgaggccggcgccaacuggaaccacuggcagcugcacgcccacuacuacccaccgcugcugagaagcgccaccgucagaaaguucauggugggauaugagaugcuggcccaggcucagagagaucugaccccggagcaggccgccgagaggcuccgcgcccucccagaagugcacuaccaucugggccagaaggacagggagacggccaccaucgcc

SEQ ID NO: 121 - RNA, 1137 nt, Artificial Sequence
  GALT-CO34
augagccggagcggcaccgacccgcagcagcgucagcaagccagcgaggccgacgccgccgccgccacguuccgggccaacgaccaccagcacauuagguacaacccgcuccaggacgaguggguccucgugagcgcccacaggaugaagaggccauggcagggacaaguugagccacagcugcugaagaccgugccacggcacgacccgcucaacccucugugcccgggcgccauccgcgccaacggcgaggugaacccacaguacgacagcaccuuccuguucgacaacgacuucccugcccuccagccggacgccccgagcccuggaccguccgaccauccgcuguuccaggccaaguccgcgcggggcgugugcaaggugaugugcuuccauccguggagcgacgugacccugccgcugauguccgugccugagauacgggccgugguggacgccugggccagcgugacagaggagcucggcgcccaguacccuugggugcagaucuucgagaacaagggugccaugauggguugcagcaacccgcacccgcauugccaggugugggccagcagcuuccugccugacaucgcccagcgggaggagcgcagccagcaggcuuacaagagccagcacggcgagccgcugcugauggaguacucuaggcaggagcugcugagaaaggagaggcuggugcugaccagcgaacacuggcucgugcuggugccguucugggcaaccuggccguaccagacccugcugcugccgaggcggcaugugagaaggcucccggagcugaccccagccgagcgcgacgaccucgccagcaucaugaagaagcuccugaccaaguacgacaaccuguucgagacgagcuucccguauuccaugggcuggcacggagccccgacaggcagcgaggccggcgccaacuggaaucacuggcagcugcaugcccacuacuacccgccgcuccugcggagcgccaccguccgcaaguucauggugggcuacgagaugcuggcccaggcccagagggaccucaccccggagcaggccgccgagaggcugcgggcccugccggagguccacuaccaccucggccagaaggauagagaaaccgccacgaucgcg

SEQ ID NO: 122 - RNA, 1137 nt, Artificial Sequence
  GALT-CO35
augagcaggagcggcaccgacccucagcagaggcaacaggccuccgaggccgacgcggcggccgccaccuucagggccaacgaccaccagcacauccgauacaacccgcuccaagacgagugggugcucgucuccgcccaccgcaugaagcggccguggcaaggucaaguugaaccacagcugcugaagaccgugccgaggcacgauccgcugaacccgcugugcccgggagccauccgggccaacggcgaggugaacccucaguacgacagcacauuccuguucgacaacgacuucccggcccugcagccggacgccccaagcccgggcccaagcgaccauccgcuguuccaagccaaguccgcccgcggcgugugcaaggugaugugcuuccacccgugguccgacgugacccugccgcugaugagcgugccggagauccgggccgugguggaugccugggccagcgugaccgaggaauuaggcgcccaguacccaugggugcagaucuucgagaacaagggagccaugaugggcugcagcaacccgcacccgcacugccaagugugggccagcuccuuccugccggacaucgcccagcgcgaggagcggagccagcaggccuacaagagucagcacggcgagccgcugcugauggaguacucuaggcaggagcugcucaggaaggagaggcuggugcugaccagcgagcacugguuggugcuggugccuuucugggccaccuggccauaccagacccugcugcugccgagaaggcacgucagaagacugccggaacugaccccggccgagagggacgaccuggccuccauuaugaagaagcuccugaccaaguacgacaaucuguucgagacguccuucccuuacagcauggguuggcacggcgccccgaccggcagcgaggcaggagccaacuggaaccacuggcagcugcacgcccacuacuacccgccgcugcucagguccgccaccguucggaaguucauggugggcuacgaaaugcuggcccaggcccagcgcgaccucaccccagagcaggccgccgagcggcugcgggcccugccggaggugcacuaccaccugggccagaaggaccgcgagacagccaccaucgcu

SEQ ID NO: 123 - RNA, 1137 nt, Artificial Sequence
  GALT-CO36
augagcaggucaggaaccgacccgcagcagcgccaacaggccuccgaggccgacgccgccgccgcgaccuuccgagccaacgaccaucaacacaucagguauaacccguugcaggacgagugggugcucguguccgcccaucggaugaagcggccguggcagggacagguggagccgcagcugcucaagaccguuccgcgccacgacccgcucaacccgcuguguccgggcgccauccgggccaacggcgaggugaacccgcaguacgacagcaccuuccuguucgacaacgauuucccugcccugcagccagaugccccgagcccgggcccuagcgaucacccgcuguuccaggccaagagcgcccggggcgucuguaaggugaugugcuuccacccauggagcgacgucacccugccgcugauguccgugccagagauccgcgccgugguggacgccugggcgagcgugaccgaggagcugggagcccaauacccuugggugcagaucuucgagaauaagggcgcuaugaugggcugcuccaacccgcacccgcacugccaggugugggccagcuccuuccucccggauaucgcccagcgggaggagagaagccagcaggccuacaagucccagcacggcgagccgcugcucauggaguauuccaggcaggagcuccucaggaaggaaaggcuugugcugacgagcgagcacuggcuggugcuggugccguucugggccaccuggccguaccagacccuccugcugccgcgccgacacgucaggaggcugccggagcugaccccggccgagagggaugaccuggccuccauaaugaagaaguuacugacuaaguaugacaacuuguucgaaaccagcuucccuuacagcaugggcuggcauggcgccccgaccggcuccgaagccggcgccaacuggaaccauuggcaacuccacgcccacuacuacccgccgcucuuaaggagcgccaccgugaggaaguucauggugggauacgagaugcuggcccaggcccaaagggaccucaccccggagcaggccgcggagaggcugcgugcccugccugagguccacuaccaccugggccagaaggacagggaaaccgcgaccaucgcc

SEQ ID NO: 124 - RNA, 1137 nt, Artificial Sequence
  GALT-CO37
augagccggagcggcaccgacccccagcagcggcagcaggccagcgaggccgacgcugccgccgccaccuuccgggccaacgaccaccagcacauccgguacaacccccugcaggacgagugggugcuggugagcgcccaccggaugaagcggcccuggcagggccagguggagccccagcugcugaagaccgugccccggcacgacccccugaacccucugugcccaggagccauccgcgccaacggcgaggugaauccucaguacgacagcaccuuccuguucgacaacgacuuccccgcccugcagcccgacgcccccagccccggccccagcgaccauccauuauuccaggccaagagcgcccggggcgugugcaaggugaugugcuuccaccccuggagcgacgugacccugccccugaugagcgugcccgagaucagagccgugguggacgccugggccagcgugaccgaggagcugggcgcccaguaccccugggugcagaucuucgagaacaagggcgccaugaugggcugcagcaacccccacccccacugccaggugugggccucaagcuuccugcccgacaucgcccagcgggaggagcggagccaacaggccuacaagucacagcacggcgagccccugcugauggaguacagccggcaggagcugcugcggaaggagcggcuggugcugaccagcgagcacuggcucgugcucgugcccuucugggccaccuggcccuaccagacccugcugcugccuagacggcacgugcggcggcugcccgagcugacccccgccgagcgggacgaccuggccagcaucaugaagaagcuccugaccaaguacgauaacuuauucgaaacaagcuuccccuacagcaugggcuggcacggcgcccccaccggcucagaggccggcgcuaacuggaaccacuggcagcugcacgcccacuacuacccgccucugcugagaagcgccaccgugcggaaguucauggugggcuacgagaugcuggcccaggcccagagagacuuaaccccugagcaggccgccgagaggcuccgggccuugccagaggugcacuaccaccugggacagaaggaccgggagacggccaccaucgcc

SEQ ID NO: 125 - RNA, 1137 nt, Artificial Sequence
  GALT-CO38
augagccggagcggcaccgacccccagcagcggcagcaggccagcgaggccgacgcagccgccgcuaccuuccgggccaacgaccaccagcacauccgguacaacccccugcaggacgagugggugcuggugagcgcccaccggaugaagcggcccuggcagggccagguggagccccagcugcugaagaccgugccccggcacgacccccugaauccucugugcccaggagccaucagagccaacggcgaggugaacccucaguacgacagcaccuuccuguucgacaacgacuuccccgcccugcagcccgacgcccccagccccggccccagcgaccauccgcuguuccaggccaagagcgcccggggcgugugcaaggugaugugcuuccaccccuggagcgacgugacccugccccugaugagcgugcccgagauccgagccgugguggacgccugggccagcgugaccgaggagcugggcgcccaguaccccugggugcagaucuucgagaacaagggcgccaugaugggcugcagcaacccccacccccacugccaggugugggccucgagcuuccugcccgacaucgcccagcgggaggagcggagccagcaagcauacaagucacagcacggcgagccccugcugauggaguacagccggcaggagcugcugcggaaggagcggcuggugcugaccagcgagcacuggcugguccuggugcccuucugggccaccuggcccuaccagacccugcuguugccuagacggcacgugcggcggcugcccgagcugacccccgccgagcgggacgaccuggccagcaucaugaagaaguugcugacaaaguaugacaaucuguucgaaaccagcuuccccuacagcaugggcuggcacggcgcccccaccggcagcgaagccggcgccaacuggaaccacuggcagcugcacgcccacuacuacccuccucugcuccgcagcgccaccgugcggaaguucauggugggcuacgagaugcuggcccaggcacagcgggaccugaccccugagcaggccgcugagagacugcgggcccucccggaggugcacuaccaccucggccagaaggaccgggaaacggccaccaucgcc

SEQ ID NO: 126 - RNA, 1137 nt, Artificial Sequence
  GALT-CO39
augagccggagcggcaccgacccccagcagcggcagcaggccagcgaggccgacgcagccgccgcgaccuuccgggccaacgaccaccagcacauccgguacaacccccugcaggacgagugggugcuggugagcgcccaccggaugaagcggcccuggcagggccagguggagccccagcugcugaagaccgugccccggcacgacccccugaacccucugugcccaggagccauuagagccaauggcgaggugaacccacaguacgacagcaccuuccuguucgacaacgacuuccccgcccugcagcccgacgcccccagccccggccccagcgaccacccgcuuuuccaggccaagagcgcccggggcgugugcaaggugaugugcuuccaccccuggagcgacgugacccugccccugaugagcgugcccgagaucagagccgugguggacgccugggccagcgugaccgaggagcugggcgcccaguaccccugggugcagaucuucgagaacaagggcgccaugaugggcugcagcaacccccacccccacugccaggugugggccucuagcuuccugcccgacaucgcccagcgggaggagcggagccagcaagccuacaagucucagcacggcgagccccugcugauggaguacagccggcaggagcugcugcggaaggagcggcuggugcugaccagcgagcacuggcugguccucgugcccuucugggccaccuggcccuaccagacccugcugcucccuagacggcacgugcggcggcugcccgagcugacccccgccgagcgggacgaccuggccagcaucaugaagaagcugcucaccaaguaugauaaucuguucgagacaagcuuccccuacagcaugggcuggcacggcgcccccaccgguucagaggccggcgccaacuggaaccacuggcagcugcacgcccacuacuacccaccuuuguugcguagcgccaccgugcggaaguucauggugggcuacgagaugcuggcccaggcccagcgcgaucugaccccagagcaggccgccgagaggcugcgggccuuaccugaggugcacuaccaccucggccagaaggaccgggaaaccgccaccaucgcc

SEQ ID NO: 127 - RNA, 1137 nt, Artificial Sequence
  GALT-CO40
augagccggagcggcaccgacccccagcagcggcagcaggccagcgaggccgacgccgcagccgcuaccuuccgggccaacgaccaccagcacauccgguacaacccccugcaggacgagugggugcuggugagcgcccaccggaugaagcggcccuggcagggccagguggagccccagcugcugaagaccgugccccggcacgacccccugaauccucucugcccuggagccauuagagccaacggcgaggugaacccacaguacgacagcaccuuccuguucgacaacgacuuccccgcccugcagcccgacgcccccagccccggccccagcgaccacccucuguuccaggccaagagcgcccggggcgugugcaaggugaugugcuuccacccauggagcgacgugacccugccccugaugagcgugcccgagaucagagcugugguggacgccugggccagcgugaccgaggagcugggcgcccaguaccccugggugcagaucuucgagaacaagggcgccaugaugggcugcagcaacccccacccccacugccaggugugggcuucuagcuuccugcccgacaucgcccagcgggaggagcggagccagcaggcguacaagucccagcacggcgagccccugcugauggaguacagccggcaggagcugcugcggaaggagcggcuggugcugaccagcgagcacuggcucguguuagugcccuucugggccaccuggcccuaccagacccugcugcugccucgucggcacgugcggcggcugcccgagcugacccccgccgagcgggacgaccuggccagcaucaugaagaagcuccugacaaaguaugacaaccuauucgaaaccagcuuccccuacagcaugggcuggcacggcgcccccaccggcagcgaagccggcgccaacuggaaccacuggcagcugcacgcccacuacuauccaccucugcugcgcagcgccaccgugcggaaguucauggugggcuacgagaugcuggcccaggcccagcgcgaccugaccccugagcaggcugccgaacgacugcgggcccugccagaagugcacuaccaccucggccagaaggaccgggagacugccaccaucgcc

SEQ ID NO: 128 - RNA, 1137 nt, Artificial Sequence
  GALT-CO41
augagccggagcggcaccgacccccagcagcggcagcaggccagcgaggccgacgcugcagccgccaccuuccgggccaacgaccaccagcacauccgguacaacccccugcaggacgagugggugcuggugagcgcccaccggaugaagcggcccuggcagggccagguggagccccagcugcugaagaccgugccccggcacgacccccugaacccucugugcccuggugccauccgagccaacggcgaggugaacccacaguacgacagcaccuuccuguucgacaacgacuuccccgcccugcagcccgacgcccccagccccggccccagcgaccauccucuguuccaggccaagagcgcccggggcgugugcaaggugaugugcuuccaccccuggagcgacgugacccugccccugaugagcgugcccgagaucagagcagugguggacgccugggccagcgugaccgaggagcugggcgcccaguaccccugggugcagaucuucgagaacaagggcgccaugaugggcugcagcaacccccacccccacugccaggugugggcuagcagcuuccugcccgacaucgcccagcgggaggagcggagccagcaggcuuacaagucucagcacggcgagccccugcugauggaguacagccggcaggagcugcugcggaaggagcggcuggugcugaccagcgagcacugguuagucuuggugcccuucugggccaccuggcccuaccagacccugcugcugccaagacggcacgugcggcggcugcccgagcugacccccgccgagcgggacgaccuggccagcaucaugaagaagcuccugacaaaguacgauaaccuuuucgagacaagcuuccccuacagcaugggcuggcacggcgccccaaccggcuccgaggccggcgcuaacuggaaccacuggcagcugcacgcccacuacuacccuccucuuuugagaagcgccaccgugcggaaguucauggugggcuacgagaugcuggcccaggcccagagggaccugaccccugagcaggccgccgagagauuacgggcucucccagaggugcacuaccaccugggacagaaggaccgggagacagccaccaucgcc

SEQ ID NO: 129 - RNA, 1137 nt, Artificial Sequence
  GALT-CO42
augagccggagcggcaccgacccccagcagcggcagcaggccagcgaggccgacgccgccgccgccaccuuccgggccaacgaccaccagcacauccgguacaacccccugcaggacgagugggugcuggugagcgcccaccggaugaagcggcccuggcagggccagguggagccccagcugcugaagaccgugccccggcacgacccccugaacccccugugccccggcgccauccgggccaacggcgaggugaacccccaguacgacagcaccuuccuguucgacaacgacuuccccgcccugcagcccgacgcccccagccccggccccagcgaccacccccuguuccaggccaagagcgcccggggcgugugcaaggugaugugcuuccaccccuggagcgacgugacccugccccugaugagcgugcccgagauccgggccgugguggacgccugggccagcgugaccgaggagcugggcgcccaguaccccugggugcagaucuucgagaacaagggcgccaugaugggcugcagcaacccccacccccacugccaggugugggccagcagcuuccugcccgacaucgcccagcgggaggagcggagccagcaggccuacaagagccagcacggcgagccccugcugauggaguacagccggcaggagcugcugcggaaggagcggcuggugcugaccagcgagcacuggcuggugcuggugcccuucugggccaccuggcccuaccagacccugcugcugccccggcggcacgugcggcggcugcccgagcugacccccgccgagcgggacgaccuggccagcaucaugaagaagcugcugaccaaguacgacaaccuguucgagaccagcuuccccuacagcaugggcuggcacggcgcccccaccggcagcgaggccggcgccaacuggaaccacuggcagcugcacgcccacuacuacccgccccugcugcggagcgccaccgugcggaaguucauggugggcuacgagaugcuggcccaggcccagcgggaccugacccccgagcaggccgccgagcggcugcgggcccugcccgaggugcacuaccaccugggccagaaggaccgggagaccgccaccaucgcc

SEQ ID NO: 130 - RNA, 1137 nt, Artificial Sequence
  GALT-CO43
augagccggagcggcaccgacccccagcagcggcagcaggccagcgaggccgacgccgccgccgccaccuuccgggccaacgaccaccagcacaucagguacaacccgcugcaggacgagugggugcuggugagcgcgcacaggaugaagaggccguggcaggggcagguggagccgcagcugcugaagacggugccgaggcacgacccgcugaacccgcugugcccgggggcgaucagggcgaacggggaggugaacccgcaguacgacagcacguuccuguucgacaacgacuucccggcgcugcagccggacgcgccgagcccggggccgagcgaccacccgcuguuccaggcgaagagcgcgaggggggugugcaaggugaugugcuuccacccguggagcgacgugacgcugccgcugaugagcgugccggagaucagggcggugguggacgcgugggcgagcgugacggaggagcugggggcgcaguacccgugggugcagaucuucgagaacaagggggcgaugauggggugcagcaacccgcacccgcacugccaggugugggcgagcagcuuccugccggacaucgcgcagagggaggagaggagccagcaggcguacaagagccagcacggggagccgcugcugauggaguacagcaggcaggagcugcugaggaaggagaggcuggugcugacgagcgagcacuggcuggugcuggugccguucugggcgacguggccguaccagacgcugcugcugccgaggaggcacgugaggaggcugccggagcugacgccggcggagagggacgaccuggcgagcaucaugaagaagcugcugacgaaguacgacaaccuguucgagacgagcuucccguacagcaugggguggcacggggcgccgacggggagcgaggcgggggcgaacuggaaccacuggcagcugcacgcgcacuacuacccgccgcugcugaggagcgcgacggugaggaaguucauggugggguacgagaugcuggcgcaggcgcagagggaccugacgccggagcaggcggcggagaggcugagggcgcugccggaggugcacuaccaccuggggcagaaggacagggagacggcgacgaucgcg

SEQ ID NO: 131 - RNA, 1137 nt, Artificial Sequence
  GALT-CO44
augagccggagcggcaccgacccccagcagcggcagcaggccagcgaggccgacgccgccgccgccaccuuccgggccaacgaccaccagcacauccgcuacaacccccuccaggacgaguggguccucgucuccgcccaccgcaugaagcgccccuggcagggccaggucgagccccagcuccucaagaccgucccccgccacgacccccucaacccccucugccccggcgccauccgcgccaacggcgaggucaacccccaguacgacuccaccuuccucuucgacaacgacuuccccgcccuccagcccgacgcccccucccccggccccuccgaccacccccucuuccaggccaaguccgcccgcggcgucugcaaggucaugugcuuccaccccugguccgacgucacccucccccucauguccguccccgagauccgcgccgucgucgacgccugggccuccgucaccgaggagcucggcgcccaguaccccuggguccagaucuucgagaacaagggcgccaugaugggcugcuccaacccccacccccacugccaggucugggccuccuccuuccuccccgacaucgcccagcgcgaggagcgcucccagcaggccuacaagucccagcacggcgagccccuccucauggaguacucccgccaggagcuccuccgcaaggagcgccucguccucaccuccgagcacuggcucguccucguccccuucugggccaccuggcccuaccagacccuccuccucccccgccgccacguccgccgccuccccgagcucacccccgccgagcgcgacgaccucgccuccaucaugaagaagcuccucaccaaguacgacaaccucuucgagaccuccuuccccuacuccaugggcuggcacggcgcccccaccggcuccgaggccggcgccaacuggaaccacuggcagcuccacgcccacuacuacccgccccuccuccgcuccgccaccguccgcaaguucauggucggcuacgagaugcucgcccaggcccagcgcgaccucacccccgagcaggccgccgagcgccuccgcgcccuccccgagguccacuaccaccucggccagaaggaccgcgagaccgccaccaucgcc

SEQ ID NO: 132 - RNA, 1348 nt, Artificial Sequence
  #1
gggaaauaagagagaaaagaagaguaagaagaaauauaagagccaccaugucuaggagcgggaccgacccccagcagcggcagcaggccagcgaggccgacgccgccgcggccaccuucagggccaacgaccaucaacacaucagguauaacccccuccaggacgaguggguguugguguccgcccaucggaugaagaggcccuggcagggccagguggagccccagcuccugaagaccgugccccggcacgacccccucaacccccugugccccggcgcgauccgcgccaacggcgaggugaacccccaguaugacagcacguuccuguucgacaacgacuuccccgcccugcagcccgacgcccccagccccggcccaagcgaccauccccuguuccaggccaaguccgccaggggcguguguaaggugaugugcuuccacccaugguccgacgugacccugccccugaugagcgugcccgagauccgcgccgugguggacgccugggccagcgugaccgaggagcugggggcccaguacccuugggugcaaaucuucgagaauaagggcgccaugaugggcugcuccaacccccacccccacugucaggugugggccagcaguuuccugcccgacaucgcccagcgcgaggagcggucacagcaggccuacaagagccaacacggcgaaccucugcucauggaguacagcaggcaggaacugcugcggaaggagaggcugguccugaccagcgagcacuggcuggugcuggugcccuucugggccaccuggcccuaccagacacugcugcugccuaggcgacacgugcgucggcugcccgagcugaccccugccgaaagggacgaccuggccagcaucaugaagaagcugcucaccaaguacgacaaccuguuugaaaccagcuuccccuacagcaugggcuggcacggcgcaccuaccggcagcgaggccggcgccaacuggaaccacuggcagcugcaugcccacuacuauccgccccuccucaggagcgccaccgugcgcaaguucauggugggcuaugagaugcuggcgcaggcccagcgugaccugacccccgagcaggccgccgagaggcugcgugcccugccugaggugcacuaccaccuggggcagaaggacagagaaacugcgaccaucgccugauaauaguccauaaaguaggaaacacuacagcuggagccucgguggccaugcuucuugccccuugggccuccccccagccccuccuccccuuccugcacccguaccccccgcauuauuacucacgguacgaguggucuuugaauaaagucugagugggcggc

SEQ ID NO: 133 - RNA, 1348 nt, Artificial Sequence
  #2
gggaaauaagagagaaaagaagaguaagaagaaauauaagagccaccaugagcagguccggcaccgacccccagcagaggcagcaagccuccgaggccgacgccgccgcggccaccuuccgggccaacgaccaucagcauaucagguauaacccccuucaggacgagugggugcucgugagcgcccaccggaugaagcgccccuggcaggggcaggucgagccccagcugcugaagaccgugcccaggcacgauccgcugaacccgcugugccccggggccauccgggccaacggggaggugaacccccaguacgacagcaccuuccuguucgacaacgacuuccccgcccugcagcccgaugcccccagccccgggcccuccgaccacccccuguuccaggccaagagcgccagaggcgugugcaaggucaugugcuuucaucccuggagcgacgugacccugccccugauguccgugcccgagaucagagcugucguggacgccugggccuccgugaccgaggagcucggcgcccaguaccccugggugcagaucuucgagaacaaaggcgccaugaugggcugcagcaacccccacccacacugccaggugugggccagcagcuuccugcccgacaucgcccagagagaggagaggagccagcaggccuauaagagccagcauggcgagccccugcugauggaguacagcagacaggagcugcugaggaaagagaggcuggugcugacaagcgagcacuggcuggugcuggugcccuuuugggccacuuggccauaccagacccugcugcugccccggcggcaugucaggagacugccugagcugacucccgccgagcgggaugaccuggccagcaucaugaagaagcugcucaccaaauacgacaaccucuucgaaaccagcuuccccuacagcaugggguggcacggggcccccaccggcagcgaagccggagccaauuggaaucauuggcagcuccaugcccauuacuauccgccccugcucagaagcgccaccgugcggaaguucauggugggcuacgagaugcucgcccaggcccagcgggaccugacccccgagcaggcugccgagcggcugagggcccugcccgaggugcacuaucaccugggccagaaagauagggaaacagccacuaucgccugauaauaguccauaaaguaggaaacacuacagcuggagccucgguggccaugcuucuugccccuugggccuccccccagccccuccuccccuuccugcacccguaccccccgcauuauuacucacgguacgaguggucuuugaauaaagucugagugggcggc

SEQ ID NO: 134 - RNA, 1348 nt, Artificial Sequence
  #3
gggaaauaagagagaaaagaagaguaagaagaaauauaagagccaccaugagcaggagcggcaccgacccccagcagaggcagcaggccagcgaagccgacgccgccgccgccaccuuccgggccaacgaucaccagcacauccgcuacaacccucuccaggacgagugggugcucgugagcgcccacaggaugaagcggcccuggcagggccagguggagccccagcuccugaagaccgugcccagacacgacccccugaacccgcucugccccggcgccaucagagccaacggcgaggugaacccccaguacgacagcaccuuccuguucgacaacgacuuccccgcccuccagcccgaugcccccagccccggucccuccgaccauccccuguuccaggccaaguccgccagaggcgugugcaaggugaugugcuuccaccccuggagcgacgugacccucccccugaugucggugcccgaaaucagggccgugguggacgccugggccagcgugaccgaggagcugggggcccaguaucccuggguccagaucuucgagaacaagggggccaugaugggcuguagcaacccccacccacacugccaggugugggccuccuccuuccugcccgacaucgcccaaagggaggagcggucccagcaagccuacaagucccagcacggugagccccugcugauggaauauagcagacaggagcugcugaggaaggagcgccugguccugaccagcgagcacuggcuggugcugguccccuuuugggccaccuggcccuaccagacgcugcugcugccucgcagacaugugaggaggcugccggagcugacccccgccgagcgggacgaccuggcaagcaucaugaagaagcugcugaccaaguacgacaaccuguucgagacuuccuucccguacagcaugggcuggcacggcgccccgaccggaagcgaggccggcgcgaacuggaaccacuggcagcugcaugcgcauuacuacccgccccugcugcggucagccaccguccgcaaguucauggugggcuacgaaaugcuggcccaggcgcagagggaccucacccccgagcaggccgccgaaagacugcgugcgcugccggaggugcacuaccaccugggccagaaggaccgcgaaaccgcgaccaucgcaugauaauaguccauaaaguaggaaacacuacagcuggagccucgguggccaugcuucuugccccuugggccuccccccagccccuccuccccuuccugcacccguaccccccgcauuauuacucacgguacgaguggucuuugaauaaagucugagugggcggc

SEQ ID NO: 135 - RNA, 1348 nt, Artificial Sequence
  #4
gggaaauaagagagaaaagaagaguaagaagaaauauaagagccaccaugucacggagcggcaccgacccgcagcagaggcagcaggccagcgaggcagacgccgccgccgccaccuucagggccaacgaccaucagcacaucagauacaacccccuacaggacgagugggugcucgucagcgcccacagaaugaagcggcccuggcaggggcagguggagccccagcuccugaagaccgugcccaggcacgacccccucaauccccugugcccuggcgccauuagggccaacggcgaggugaacccccaguacgacucaaccuuccuguuugacaacgacuuccccgcccugcagcccgaugccccgagccccgggcccagcgaccacccccuguuccaggccaagucggccaggggcgugugcaaggugaugugcuuccaccccuggagcgaugucacccugccccugaugucggugcccgagauccgcgccgugguggacgccugggccagcgugaccgaggagcugggcgcccaauaccccugggugcagaucuuugagaacaaaggcgccaugaugggcuguagcaacccccacccccacugucaggugugggccagcagcuuucugcccgacaucgcccagagggaggagcgcucccagcaggcuuacaagagccagcacggagagccccugcucauggaguacucgcgacaggagcugcuccggaaggaacggcugguccugaccuccgagcacuggcucgugcuggugccguucugggccacauggcccuaccagacccugcugcuaccccgcagacacguucgccgacugcccgagcugaccccugccgagagagacgaccuggcgagcaucaugaagaagcugcucaccaaguaugacaacuuauucgaaaccuccuucccuuacagcaugggcuggcacggcgcccccaccggcagcgaggcgggcgccaacuggaaccacuggcagcugcaugcccacuacuacccaccccugcugcggagcgccaccgugagaaaguucauggugggcuacgagaugcuggcccaggcccaacgggaucugacccccgagcaggccgccgagcggcugagggcccuccccgagguacacuaccaucucggccagaaggaccgggaaaccgccaccaucgccugauaauaguccauaaaguaggaaacacuacagcuggagccucgguggccaugcuucuugccccuugggccuccccccagccccuccuccccuuccugcacccguaccccccgcauuauuacucacgguacgaguggucuuugaauaaagucugagugggcggc

SEQ ID NO: 136 - RNA, 1348 nt, Artificial Sequence
  #5
gggaaauaagagagaaaagaagaguaagaagaaauauaagagccaccaugagcagaagcggcaccgacccccagcagcggcagcaggccagcgaggccgacgccgccgccgcaaccuuccgcgccaacgaccaccagcacaucagauacaacccccuccaggacgaguggguccucguguccgcccauagaaugaagaggccauggcagggccagguagaaccucaacugcugaagaccgucccccggcaugacccccucaauccccucugcccgggggccauccgagcgaauggggaggucaacccccaguacgacagcaccuuccuguucgacaacgacuuccccgcccugcagcccgacgccccgagccccggacccagcgaccacccccuguuccaggccaaauccgcccggggcgucugcaaggugaugugcuuucaccccugguccgacgugacccugccccucauguccgugcccgagaucagggccgugguggacgcuugggccagcgucacggaggagcucggcgcccaguaccccuggguccagaucuucgagaacaagggcgccaugauggggugcuccaacccucacccccacugccaggugugggccagcagcuuucugcccgacauugcccagcgggaggagaggucccagcaggccuacaagagucagcacggggagccccugcugauggaguacucccggcaggagcuccugaggaaagagcgcuuggugcugacaagcgagcacuggcuggugcucgugcccuucugggccacuuggcccuaccagacccugcugcugcccagacggcacgugcggcggcugcccgagcugacacccgccgagagggacgaucucgccagcauuaugaagaagcugcugaccaaguaugacaaccuguuugagacuagcuuucccuacagcaugggcuggcacggggcccccacgggcuccgaggccggcgccaacuggaaccacuggcagcugcacgcccacuauuauccgccccugcuccggagcgccaccgugagaaaguuuauggugggcuaugagaugcuggcccaagcgcaacgggaucugacccccgagcaggccgccgagcgucugagagcccugccugaggugcacuaucaccuggggcagaaggaccgggagacggcaaccaucgccugauaauaguccauaaaguaggaaacacuacagcuggagccucgguggccaugcuucuugccccuugggccuccccccagccccuccuccccuuccugcacccguaccccccgcauuauuacucacgguacgaguggucuuugaauaaagucugagugggcggc

SEQ ID NO: 137 - RNA, 1348 nt, Artificial Sequence
  #6
gggaaauaagagagaaaagaagaguaagaagaaauauaagagccaccaugagccgcagcggcaccgacccgcaacaaagacagcaggccuccgaggccgacgccgccgccgcuaccuuuagggccaacgaccaccagcauauccgcuacaauccccuccaggacgagugggugcucgugagcgcccaccguaugaagaggcccuggcagggacagguggaaccccagcugcugaagaccguaccccggcacgacccccugaacccccugugccccggggccaucagagccaauggagaggugaacccccaguacgacuccaccuuccuguucgauaaugauuuuccggcccugcagcccgacgcccccagccccggcccaagcgaccacccucuguuccaggccaagagcgccaggggcguuugcaaggucaugugcuuccaccccuggagcgacgugacccugccccugaugucggugcccgagaucagggccgugguggacgccugggccagcgugacggaggaacucggcgcccaguaccccuggguacagaucuucgagaacaagggugccaugaugggcugcagcaacccacauccccacugucaggugugggccagcucauuccugccugacaucgcccagcgugaggagaggagucagcaggccuauaagagccagcauggggagccccuccugauggaguacagcagacaagagcugcucaggaaggagagacuggugcugaccagcgagcauuggcuggugcuggugcccuuuugggccacauggcccuaccagacccuccugcugccgagacgccacgugcgccggcugcccgagcugacucccgccgagagggacgaccucgcuagcaucaugaagaaacugcugaccaaguacgacaaccuguuugagacaagcuuucccuacuccaugggauggcacggcgcccccaccggcuccgaggccggcgccaacuggaaccacuggcagcugcacgcccacuacuaucccccgcugcugcggagcgccaccgugaggaaauucauggugggcuacgagaugcucgcucaggcccaacgggaccugacccccgagcaggcggccgagaggcuccgagcucugcccgaggugcauuaccaucugggccagaaggauagggaaaccgccaccaucgccugauaauaguccauaaaguaggaaacacuacagcuggagccucgguggccaugcuucuugccccuugggccuccccccagccccuccuccccuuccugcacccguaccccccgcauuauuacucacgguacgaguggucuuugaauaaagucugagugggcggc

SEQ ID NO: 138 - RNA, 1348 nt, Artificial Sequence
  #7
gggaaauaagagagaaaagaagaguaagaagaaauauaagagccaccaugagcaggagcggaaccgacccgcagcagaggcagcaggccagcgaagccgacgccgccgccgccaccuuccgggccaacgaccaccaacacaucagguacaacccgcuccaggacgagugggugcucguuagcgcccaucgcaugaagcggccguggcaaggccagguggagccgcagcugcugaagaccgugccgcgccacgacccgcugaacccgcugugcccuggcgccauccgggccaacggcgaggugaacccucaguacgacagcaccuuccuguucgacaaugauuucccggccuugcagccggacgccccuuccccgggaccguccgaccacccgcuguuccaagccaaguccgcccggggcgugugcaaggugaugugcuuccacccgugguccgacgugacccugccgcugaugagcgugccugagaucagagccgugguggacgccugggccuccgugacugaggagcucggcgcccaguacccauggguccagaucuucgagaacaagggugccaugaugggcugcagcaacccgcacccgcacugccaagugugggccagcuccuuccugccggauauugcccagcgggaggagcggagccagcaagcauacaagagccagcauggcgagccgcucuugauggaguacuccaggcaggagcugcugagaaaggagcggcuggugcugaccucugagcacuggcuggugcucgugccguucugggccaccuggccuuaccagacccugcugcugccgaggcggcacgugcgccggcugccagagcugacgccagccgagcgagacgaucuggccuccaucaugaagaagcuacugaccaaguaugacaaccuguucgaaacgagcuucccguacagcaugggcuggcacggcgccccgaccggcagcgaggccggcgccaacuggaaucacuggcagcugcaugcccauuacuacccgccgcuccuccgcagcgccaccgugaggaaguucauggugggcuacgagaugcuggcccaggcccagcgggaccugaccccggagcaggcggccgagagacugagggcccucccggagguccauuaccaccugggccagaaggaccgggagacggccaccaucgccugauaauaguccauaaaguaggaaacacuacagcuggagccucgguggccaugcuucuugccccuugggccuccccccagccccuccuccccuuccugcacccguaccccccgcauuauuacucacgguacgaguggucuuugaauaaagucugagugggcggc

SEQ ID NO: 139 - RNA, 1348 nt, Artificial Sequence
  #8
gggaaauaagagagaaaagaagaguaagaagaaauauaagagccaccaugucccgcagcggcacggacccgcagcagcggcagcaggccagcgaggccgacgccgcggccgccaccuuccgggccaacgaccaccagcacaucagguacaacccacuccaagacgagugggugcucgugagcgcccaccggaugaagaggccguggcagggacagguugagccgcaacugcugaagaccgugccaagacacgauccgcugaacccgcucugcccgggcgccauccgugccaacggcgaggucaacccacaguaugacagcaccuuccuguucgacaacgacuucccggcccugcagccggacgcgccuagcccuggaccguccgaccacccgcuguuccaggccaaguccgcuaggggcgugugcaaggugaugugcuuccauccgugguccgaugucacccugccgcucauguccgugccggagauccgggccgugguggaugccugggccagcgucaccgaggagcugggcgcgcaguacccuuggguccagaucuucgagaacaagggcgccaugauggguugcagcaacccgcacccacacugccaggugugggccagcagcuuccugccggacaucgcacagagggaggagcggagccaacaggccuacaagucccagcacggcgagccacugcugauggaguacagcaggcaggagcugcugcggaaggagcggcuggugcucaccuccgaacauuggcugguucuggugccguucugggccaccuggccuuaccagacccugcugcucccgaggcggcacgugcgcaggcugccggagcugacaccggccgagcgcgacgaccuggccagcaucaugaagaagcugcucaccaaguacgauaaccuguucgagacauccuucccguacagcaugggcuggcacggcgccccuaccggcuccgaggccggcgccaacuggaaccacuggcagcugcacgcccacuacuacccaccgcugcugagaagcgccaccgucagaaaguucauggugggauaugagaugcuggcccaggcucagagagaucugaccccggagcaggccgccgagaggcuccgcgcccucccagaagugcacuaccaucugggccagaaggacagggagacggccaccaucgccugauaauaguccauaaaguaggaaacacuacagcuggagccucgguggccaugcuucuugccccuugggccuccccccagccccuccuccccuuccugcacccguaccccccgcauuauuacucacgguacgaguggucuuugaauaaagucugagugggcggc

SEQ ID NO: 140 - RNA, 1348 nt, Artificial Sequence
  #9
gggaaauaagagagaaaagaagaguaagaagaaauauaagagccaccaugagccggagcggcaccgacccgcagcagcgucagcaagccagcgaggccgacgccgccgccgccacguuccgggccaacgaccaccagcacauuagguacaacccgcuccaggacgaguggguccucgugagcgcccacaggaugaagaggccauggcagggacaaguugagccacagcugcugaagaccgugccacggcacgacccgcucaacccucugugcccgggcgccauccgcgccaacggcgaggugaacccacaguacgacagcaccuuccuguucgacaacgacuucccugcccuccagccggacgccccgagcccuggaccguccgaccauccgcuguuccaggccaaguccgcgcggggcgugugcaaggugaugugcuuccauccguggagcgacgugacccugccgcugauguccgugccugagauacgggccgugguggacgccugggccagcgugacagaggagcucggcgcccaguacccuugggugcagaucuucgagaacaagggugccaugauggguugcagcaacccgcacccgcauugccaggugugggccagcagcuuccugccugacaucgcccagcgggaggagcgcagccagcaggcuuacaagagccagcacggcgagccgcugcugauggaguacucuaggcaggagcugcugagaaaggagaggcuggugcugaccagcgaacacuggcucgugcuggugccguucugggcaaccuggccguaccagacccugcugcugccgaggcggcaugugagaaggcucccggagcugaccccagccgagcgcgacgaccucgccagcaucaugaagaagcuccugaccaaguacgacaaccuguucgagacgagcuucccguauuccaugggcuggcacggagccccgacaggcagcgaggccggcgccaacuggaaucacuggcagcugcaugcccacuacuacccgccgcuccugcggagcgccaccguccgcaaguucauggugggcuacgagaugcuggcccaggcccagagggaccucaccccggagcaggccgccgagaggcugcgggcccugccggagguccacuaccaccucggccagaaggauagagaaaccgccacgaucgcgugauaauaguccauaaaguaggaaacacuacagcuggagccucgguggccaugcuucuugccccuugggccuccccccagccccuccuccccuuccugcacccguaccccccgcauuauuacucacgguacgaguggucuuugaauaaagucugagugggcggc

SEQ ID NO: 141 - RNA, 1348 nt, Artificial Sequence
  #10
gggaaauaagagagaaaagaagaguaagaagaaauauaagagccaccaugagcaggagcggcaccgacccucagcagaggcaacaggccuccgaggccgacgcggcggccgccaccuucagggccaacgaccaccagcacauccgauacaacccgcuccaagacgagugggugcucgucuccgcccaccgcaugaagcggccguggcaaggucaaguugaaccacagcugcugaagaccgugccgaggcacgauccgcugaacccgcugugcccgggagccauccgggccaacggcgaggugaacccucaguacgacagcacauuccuguucgacaacgacuucccggcccugcagccggacgccccaagcccgggcccaagcgaccauccgcuguuccaagccaaguccgcccgcggcgugugcaaggugaugugcuuccacccgugguccgacgugacccugccgcugaugagcgugccggagauccgggccgugguggaugccugggccagcgugaccgaggaauuaggcgcccaguacccaugggugcagaucuucgagaacaagggagccaugaugggcugcagcaacccgcacccgcacugccaagugugggccagcuccuuccugccggacaucgcccagcgcgaggagcggagccagcaggccuacaagagucagcacggcgagccgcugcugauggaguacucuaggcaggagcugcucaggaaggagaggcuggugcugaccagcgagcacugguuggugcuggugccuuucugggccaccuggccauaccagacccugcugcugccgagaaggcacgucagaagacugccggaacugaccccggccgagagggacgaccuggccuccauuaugaagaagcuccugaccaaguacgacaaucuguucgagacguccuucccuuacagcauggguuggcacggcgccccgaccggcagcgaggcaggagccaacuggaaccacuggcagcugcacgcccacuacuacccgccgcugcucagguccgccaccguucggaaguucauggugggcuacgaaaugcuggcccaggcccagcgcgaccucaccccagagcaggccgccgagcggcugcgggcccugccggaggugcacuaccaccugggccagaaggaccgcgagacagccaccaucgcuugauaauaguccauaaaguaggaaacacuacagcuggagccucgguggccaugcuucuugccccuugggccuccccccagccccuccuccccuuccugcacccguaccccccgcauuauuacucacgguacgaguggucuuugaauaaagucugagugggcggc

SEQ ID NO: 142 - RNA, 1348 nt, Artificial Sequence
  #11
gggaaauaagagagaaaagaagaguaagaagaaauauaagagccaccaugagcaggucaggaaccgacccgcagcagcgccaacaggccuccgaggccgacgccgccgccgcgaccuuccgagccaacgaccaucaacacaucagguauaacccguugcaggacgagugggugcucguguccgcccaucggaugaagcggccguggcagggacagguggagccgcagcugcucaagaccguuccgcgccacgacccgcucaacccgcuguguccgggcgccauccgggccaacggcgaggugaacccgcaguacgacagcaccuuccuguucgacaacgauuucccugcccugcagccagaugccccgagcccgggcccuagcgaucacccgcuguuccaggccaagagcgcccggggcgucuguaaggugaugugcuuccacccauggagcgacgucacccugccgcugauguccgugccagagauccgcgccgugguggacgccugggcgagcgugaccgaggagcugggagcccaauacccuugggugcagaucuucgagaauaagggcgcuaugaugggcugcuccaacccgcacccgcacugccaggugugggccagcuccuuccucccggauaucgcccagcgggaggagagaagccagcaggccuacaagucccagcacggcgagccgcugcucauggaguauuccaggcaggagcuccucaggaaggaaaggcuugugcugacgagcgagcacuggcuggugcuggugccguucugggccaccuggccguaccagacccuccugcugccgcgccgacacgucaggaggcugccggagcugaccccggccgagagggaugaccuggccuccauaaugaagaaguuacugacuaaguaugacaacuuguucgaaaccagcuucccuuacagcaugggcuggcauggcgccccgaccggcuccgaagccggcgccaacuggaaccauuggcaacuccacgcccacuacuacccgccgcucuuaaggagcgccaccgugaggaaguucauggugggauacgagaugcuggcccaggcccaaagggaccucaccccggagcaggccgcggagaggcugcgugcccugccugagguccacuaccaccugggccagaaggacagggaaaccgcgaccaucgccugauaauaguccauaaaguaggaaacacuacagcuggagccucgguggccaugcuucuugccccuugggccuccccccagccccuccuccccuuccugcacccguaccccccgcauuauuacucacgguacgaguggucuuugaauaaagucugagugggcggc

SEQ ID NO: 143 - RNA, 1348 nt, Artificial Sequence
  #12
gggaaauaagagagaaaagaagaguaagaagaaauauaagagccaccaugagccggagcggcaccgacccccagcagcggcagcaggccagcgaggccgacgcugccgccgccaccuuccgggccaacgaccaccagcacauccgguacaacccccugcaggacgagugggugcuggugagcgcccaccggaugaagcggcccuggcagggccagguggagccccagcugcugaagaccgugccccggcacgacccccugaacccucugugcccaggagccauccgcgccaacggcgaggugaauccucaguacgacagcaccuuccuguucgacaacgacuuccccgcccugcagcccgacgcccccagccccggccccagcgaccauccauuauuccaggccaagagcgcccggggcgugugcaaggugaugugcuuccaccccuggagcgacgugacccugccccugaugagcgugcccgagaucagagccgugguggacgccugggccagcgugaccgaggagcugggcgcccaguaccccugggugcagaucuucgagaacaagggcgccaugaugggcugcagcaacccccacccccacugccaggugugggccucaagcuuccugcccgacaucgcccagcgggaggagcggagccaacaggccuacaagucacagcacggcgagccccugcugauggaguacagccggcaggagcugcugcggaaggagcggcuggugcugaccagcgagcacuggcucgugcucgugcccuucugggccaccuggcccuaccagacccugcugcugccuagacggcacgugcggcggcugcccgagcugacccccgccgagcgggacgaccuggccagcaucaugaagaagcuccugaccaaguacgauaacuuauucgaaacaagcuuccccuacagcaugggcuggcacggcgcccccaccggcucagaggccggcgcuaacuggaaccacuggcagcugcacgcccacuacuacccgccucugcugagaagcgccaccgugcggaaguucauggugggcuacgagaugcuggcccaggcccagagagacuuaaccccugagcaggccgccgagaggcuccgggccuugccagaggugcacuaccaccugggacagaaggaccgggagacggccaccaucgccugauaauaguccauaaaguaggaaacacuacagcuggagccucgguggccaugcuucuugccccuugggccuccccccagccccuccuccccuuccugcacccguaccccccgcauuauuacucacgguacgaguggucuuugaauaaagucugagugggcggc

SEQ ID NO: 144 - RNA, 1348 nt, Artificial Sequence
  #13
gggaaauaagagagaaaagaagaguaagaagaaauauaagagccaccaugagccggagcggcaccgacccccagcagcggcagcaggccagcgaggccgacgcagccgccgcuaccuuccgggccaacgaccaccagcacauccgguacaacccccugcaggacgagugggugcuggugagcgcccaccggaugaagcggcccuggcagggccagguggagccccagcugcugaagaccgugccccggcacgacccccugaauccucugugcccaggagccaucagagccaacggcgaggugaacccucaguacgacagcaccuuccuguucgacaacgacuuccccgcccugcagcccgacgcccccagccccggccccagcgaccauccgcuguuccaggccaagagcgcccggggcgugugcaaggugaugugcuuccaccccuggagcgacgugacccugccccugaugagcgugcccgagauccgagccgugguggacgccugggccagcgugaccgaggagcugggcgcccaguaccccugggugcagaucuucgagaacaagggcgccaugaugggcugcagcaacccccacccccacugccaggugugggccucgagcuuccugcccgacaucgcccagcgggaggagcggagccagcaagcauacaagucacagcacggcgagccccugcugauggaguacagccggcaggagcugcugcggaaggagcggcuggugcugaccagcgagcacuggcugguccuggugcccuucugggccaccuggcccuaccagacccugcuguugccuagacggcacgugcggcggcugcccgagcugacccccgccgagcgggacgaccuggccagcaucaugaagaaguugcugacaaaguaugacaaucuguucgaaaccagcuuccccuacagcaugggcuggcacggcgcccccaccggcagcgaagccggcgccaacuggaaccacuggcagcugcacgcccacuacuacccuccucugcuccgcagcgccaccgugcggaaguucauggugggcuacgagaugcuggcccaggcacagcgggaccugaccccugagcaggccgcugagagacugcgggcccucccggaggugcacuaccaccucggccagaaggaccgggaaacggccaccaucgccugauaauaguccauaaaguaggaaacacuacagcuggagccucgguggccaugcuucuugccccuugggccuccccccagccccuccuccccuuccugcacccguaccccccgcauuauuacucacgguacgaguggucuuugaauaaagucugagugggcggc

SEQ ID NO: 145 - RNA, 1348 nt, Artificial Sequence
  #14
gggaaauaagagagaaaagaagaguaagaagaaauauaagagccaccaugagccggagcggcaccgacccccagcagcggcagcaggccagcgaggccgacgcagccgccgcgaccuuccgggccaacgaccaccagcacauccgguacaacccccugcaggacgagugggugcuggugagcgcccaccggaugaagcggcccuggcagggccagguggagccccagcugcugaagaccgugccccggcacgacccccugaacccucugugcccaggagccauuagagccaauggcgaggugaacccacaguacgacagcaccuuccuguucgacaacgacuuccccgcccugcagcccgacgcccccagccccggccccagcgaccacccgcuuuuccaggccaagagcgcccggggcgugugcaaggugaugugcuuccaccccuggagcgacgugacccugccccugaugagcgugcccgagaucagagccgugguggacgccugggccagcgugaccgaggagcugggcgcccaguaccccugggugcagaucuucgagaacaagggcgccaugaugggcugcagcaacccccacccccacugccaggugugggccucuagcuuccugcccgacaucgcccagcgggaggagcggagccagcaagccuacaagucucagcacggcgagccccugcugauggaguacagccggcaggagcugcugcggaaggagcggcuggugcugaccagcgagcacuggcugguccucgugcccuucugggccaccuggcccuaccagacccugcugcucccuagacggcacgugcggcggcugcccgagcugacccccgccgagcgggacgaccuggccagcaucaugaagaagcugcucaccaaguaugauaaucuguucgagacaagcuuccccuacagcaugggcuggcacggcgcccccaccgguucagaggccggcgccaacuggaaccacuggcagcugcacgcccacuacuacccaccuuuguugcguagcgccaccgugcggaaguucauggugggcuacgagaugcuggcccaggcccagcgcgaucugaccccagagcaggccgccgagaggcugcgggccuuaccugaggugcacuaccaccucggccagaaggaccgggaaaccgccaccaucgccugauaauaguccauaaaguaggaaacacuacagcuggagccucgguggccaugcuucuugccccuugggccuccccccagccccuccuccccuuccugcacccguaccccccgcauuauuacucacgguacgaguggucuuugaauaaagucugagugggcggc

SEQ ID NO: 146 - RNA, 1348 nt, Artificial Sequence
  #15
gggaaauaagagagaaaagaagaguaagaagaaauauaagagccaccaugagccggagcggcaccgacccccagcagcggcagcaggccagcgaggccgacgccgcagccgcuaccuuccgggccaacgaccaccagcacauccgguacaacccccugcaggacgagugggugcuggugagcgcccaccggaugaagcggcccuggcagggccagguggagccccagcugcugaagaccgugccccggcacgacccccugaauccucucugcccuggagccauuagagccaacggcgaggugaacccacaguacgacagcaccuuccuguucgacaacgacuuccccgcccugcagcccgacgcccccagccccggccccagcgaccacccucuguuccaggccaagagcgcccggggcgugugcaaggugaugugcuuccacccauggagcgacgugacccugccccugaugagcgugcccgagaucagagcugugguggacgccugggccagcgugaccgaggagcugggcgcccaguaccccugggugcagaucuucgagaacaagggcgccaugaugggcugcagcaacccccacccccacugccaggugugggcuucuagcuuccugcccgacaucgcccagcgggaggagcggagccagcaggcguacaagucccagcacggcgagccccugcugauggaguacagccggcaggagcugcugcggaaggagcggcuggugcugaccagcgagcacuggcucguguuagugcccuucugggccaccuggcccuaccagacccugcugcugccucgucggcacgugcggcggcugcccgagcugacccccgccgagcgggacgaccuggccagcaucaugaagaagcuccugacaaaguaugacaaccuauucgaaaccagcuuccccuacagcaugggcuggcacggcgcccccaccggcagcgaagccggcgccaacuggaaccacuggcagcugcacgcccacuacuauccaccucugcugcgcagcgccaccgugcggaaguucauggugggcuacgagaugcuggcccaggcccagcgcgaccugaccccugagcaggcugccgaacgacugcgggcccugccagaagugcacuaccaccucggccagaaggaccgggagacugccaccaucgccugauaauaguccauaaaguaggaaacacuacagcuggagccucgguggccaugcuucuugccccuugggccuccccccagccccuccuccccuuccugcacccguaccccccgcauuauuacucacgguacgaguggucuuugaauaaagucugagugggcggc

SEQ ID NO: 147 - RNA, 1348 nt, Artificial Sequence
  #16
gggaaauaagagagaaaagaagaguaagaagaaauauaagagccaccaugagccggagcggcaccgacccccagcagcggcagcaggccagcgaggccgacgcugcagccgccaccuuccgggccaacgaccaccagcacauccgguacaacccccugcaggacgagugggugcuggugagcgcccaccggaugaagcggcccuggcagggccagguggagccccagcugcugaagaccgugccccggcacgacccccugaacccucugugcccuggugccauccgagccaacggcgaggugaacccacaguacgacagcaccuuccuguucgacaacgacuuccccgcccugcagcccgacgcccccagccccggccccagcgaccauccucuguuccaggccaagagcgcccggggcgugugcaaggugaugugcuuccaccccuggagcgacgugacccugccccugaugagcgugcccgagaucagagcagugguggacgccugggccagcgugaccgaggagcugggcgcccaguaccccugggugcagaucuucgagaacaagggcgccaugaugggcugcagcaacccccacccccacugccaggugugggcuagcagcuuccugcccgacaucgcccagcgggaggagcggagccagcaggcuuacaagucucagcacggcgagccccugcugauggaguacagccggcaggagcugcugcggaaggagcggcuggugcugaccagcgagcacugguuagucuuggugcccuucugggccaccuggcccuaccagacccugcugcugccaagacggcacgugcggcggcugcccgagcugacccccgccgagcgggacgaccuggccagcaucaugaagaagcuccugacaaaguacgauaaccuuuucgagacaagcuuccccuacagcaugggcuggcacggcgccccaaccggcuccgaggccggcgcuaacuggaaccacuggcagcugcacgcccacuacuacccuccucuuuugagaagcgccaccgugcggaaguucauggugggcuacgagaugcuggcccaggcccagagggaccugaccccugagcaggccgccgagagauuacgggcucucccagaggugcacuaccaccugggacagaaggaccgggagacagccaccaucgccugauaauaguccauaaaguaggaaacacuacagcuggagccucgguggccaugcuucuugccccuugggccuccccccagccccuccuccccuuccugcacccguaccccccgcauuauuacucacgguacgaguggucuuugaauaaagucugagugggcggc

SEQ ID NO: 148 - RNA, 1348 nt, Artificial Sequence
  #17
gggaaauaagagagaaaagaagaguaagaagaaauauaagagccaccaugagccggagcggcaccgacccccagcagcggcagcaggccagcgaggccgacgccgccgccgccaccuuccgggccaacgaccaccagcacauccgguacaacccccugcaggacgagugggugcuggugagcgcccaccggaugaagcggcccuggcagggccagguggagccccagcugcugaagaccgugccccggcacgacccccugaacccccugugccccggcgccauccgggccaacggcgaggugaacccccaguacgacagcaccuuccuguucgacaacgacuuccccgcccugcagcccgacgcccccagccccggccccagcgaccacccccuguuccaggccaagagcgcccggggcgugugcaaggugaugugcuuccaccccuggagcgacgugacccugccccugaugagcgugcccgagauccgggccgugguggacgccugggccagcgugaccgaggagcugggcgcccaguaccccugggugcagaucuucgagaacaagggcgccaugaugggcugcagcaacccccacccccacugccaggugugggccagcagcuuccugcccgacaucgcccagcgggaggagcggagccagcaggccuacaagagccagcacggcgagccccugcugauggaguacagccggcaggagcugcugcggaaggagcggcuggugcugaccagcgagcacuggcuggugcuggugcccuucugggccaccuggcccuaccagacccugcugcugccccggcggcacgugcggcggcugcccgagcugacccccgccgagcgggacgaccuggccagcaucaugaagaagcugcugaccaaguacgacaaccuguucgagaccagcuuccccuacagcaugggcuggcacggcgcccccaccggcagcgaggccggcgccaacuggaaccacuggcagcugcacgcccacuacuacccgccccugcugcggagcgccaccgugcggaaguucauggugggcuacgagaugcuggcccaggcccagcgggaccugacccccgagcaggccgccgagcggcugcgggcccugcccgaggugcacuaccaccugggccagaaggaccgggagaccgccaccaucgccugauaauaguccauaaaguaggaaacacuacagcuggagccucgguggccaugcuucuugccccuugggccuccccccagccccuccuccccuuccugcacccguaccccccgcauuauuacucacgguacgaguggucuuugaauaaagucugagugggcggc

SEQ ID NO: 149 - RNA, 1348 nt, Artificial Sequence
  #18
gggaaauaagagagaaaagaagaguaagaagaaauauaagagccaccaugagccggagcggcaccgacccccagcagcggcagcaggccagcgaggccgacgccgccgccgccaccuuccgggccaacgaccaccagcacaucagguacaacccgcugcaggacgagugggugcuggugagcgcgcacaggaugaagaggccguggcaggggcagguggagccgcagcugcugaagacggugccgaggcacgacccgcugaacccgcugugcccgggggcgaucagggcgaacggggaggugaacccgcaguacgacagcacguuccuguucgacaacgacuucccggcgcugcagccggacgcgccgagcccggggccgagcgaccacccgcuguuccaggcgaagagcgcgaggggggugugcaaggugaugugcuuccacccguggagcgacgugacgcugccgcugaugagcgugccggagaucagggcggugguggacgcgugggcgagcgugacggaggagcugggggcgcaguacccgugggugcagaucuucgagaacaagggggcgaugauggggugcagcaacccgcacccgcacugccaggugugggcgagcagcuuccugccggacaucgcgcagagggaggagaggagccagcaggcguacaagagccagcacggggagccgcugcugauggaguacagcaggcaggagcugcugaggaaggagaggcuggugcugacgagcgagcacuggcuggugcuggugccguucugggcgacguggccguaccagacgcugcugcugccgaggaggcacgugaggaggcugccggagcugacgccggcggagagggacgaccuggcgagcaucaugaagaagcugcugacgaaguacgacaaccuguucgagacgagcuucccguacagcaugggguggcacggggcgccgacggggagcgaggcgggggcgaacuggaaccacuggcagcugcacgcgcacuacuacccgccgcugcugaggagcgcgacggugaggaaguucauggugggguacgagaugcuggcgcaggcgcagagggaccugacgccggagcaggcggcggagaggcugagggcgcugccggaggugcacuaccaccuggggcagaaggacagggagacggcgacgaucgcgugauaauaguccauaaaguaggaaacacuacagcuggagccucgguggccaugcuucuugccccuugggccuccccccagccccuccuccccuuccugcacccguaccccccgcauuauuacucacgguacgaguggucuuugaauaaagucugagugggcggc

SEQ ID NO: 150 - RNA, 1348 nt, Artificial Sequence
  #19
gggaaauaagagagaaaagaagaguaagaagaaauauaagagccaccaugagccggagcggcaccgacccccagcagcggcagcaggccagcgaggccgacgccgccgccgccaccuuccgggccaacgaccaccagcacauccgcuacaacccccuccaggacgaguggguccucgucuccgcccaccgcaugaagcgccccuggcagggccaggucgagccccagcuccucaagaccgucccccgccacgacccccucaacccccucugccccggcgccauccgcgccaacggcgaggucaacccccaguacgacuccaccuuccucuucgacaacgacuuccccgcccuccagcccgacgcccccucccccggccccuccgaccacccccucuuccaggccaaguccgcccgcggcgucugcaaggucaugugcuuccaccccugguccgacgucacccucccccucauguccguccccgagauccgcgccgucgucgacgccugggccuccgucaccgaggagcucggcgcccaguaccccuggguccagaucuucgagaacaagggcgccaugaugggcugcuccaacccccacccccacugccaggucugggccuccuccuuccuccccgacaucgcccagcgcgaggagcgcucccagcaggccuacaagucccagcacggcgagccccuccucauggaguacucccgccaggagcuccuccgcaaggagcgccucguccucaccuccgagcacuggcucguccucguccccuucugggccaccuggcccuaccagacccuccuccucccccgccgccacguccgccgccuccccgagcucacccccgccgagcgcgacgaccucgccuccaucaugaagaagcuccucaccaaguacgacaaccucuucgagaccuccuuccccuacuccaugggcuggcacggcgcccccaccggcuccgaggccggcgccaacuggaaccacuggcagcuccacgcccacuacuacccgccccuccuccgcuccgccaccguccgcaaguucauggucggcuacgagaugcucgcccaggcccagcgcgaccucacccccgagcaggccgccgagcgccuccgcgcccuccccgagguccacuaccaccucggccagaaggaccgcgagaccgccaccaucgccugauaauaguccauaaaguaggaaacacuacagcuggagccucgguggccaugcuucuugccccuugggccuccccccagccccuccuccccuuccugcacccguaccccccgcauuauuacucacgguacgaguggucuuugaauaaagucugagugggcggc

SEQ ID NO: 151 - RNA, 810 nt, Artificial Sequence
  Human GALT isoform 2
augacccucucaacccucuguguccuggggccauccgagccaacggagaguaaggucaugugcuuccaccccuggucggauguaacgcugccacucaugucggucccugagauccgggcuguuguugaugcaugggccucagucacagaggagcugggugcccaguacccuugggugcagaucuuugaaaacaaaggugccaugaugggcuguucuaacccccacccccacugccagguaugggccagcaguuuccugccagauauugcccagcgugaggagcgaucucagcaggccuauaagagucagcauggagagccccugcuaauggaguacagccgccaggagcuacucaggaaggaacgucugguccuaaccagugagcacugguuaguacugguccccuucugggcaacauggcccuaccagacacugcugcugccccgucggcaugugcggcggcuaccugagcugaccccugcugagcgugaugaucuagccuccaucaugaagaagcucuugaccaaguaugacaaccucuuugagacguccuuucccuacuccaugggcuggcauggggcucccacaggaucagaggcuggggccaacuggaaccauuggcagcugcacgcucauuacuacccuccgcuccugcgcucugccacuguccggaaauucaugguuggcuacgaaaugcuugcucaggcucagagggaccucaccccugagcaggcugcagagagacuaagggcacuuccugagguucauuaccaccuggggcagaaggacagggagacagcaaccaucgcc

SEQ ID NO: 152 - RNA, 609 nt, Artificial Sequence
  Mouse GALT isoform 2
augaugggcuguucuaacccccauccccacugccagguuugggcuagcagcuuccugccagauaucgcccagcgugaagagcgaucccagcagaccuaucacagccagcauggaaaaccuuuguuauuggaauauggucaccaagagcuccucaggaaggaacgucugguccuaaccagugagcacuggauaguucugguccccuucugggcaguguggccuuuccagacacuucugcugccccggcggcacgugcggcggcuaccugagcugaaccccgcugagcgugaugaucucgccuccaucaugaagaagcucuugaccaaguacgacaaucuauuugagacauccuuucccuacuccaugggcuggcauggggcucccacgggauuaaagacuggagccaccugugaccacuggcagcuccacgcccacuacuaccccccacuucugcgauccgcaacuguccggaaguucaugguuggcuaugaaaugcuugcccaggcccagcgugaccucacucccgaacaggccgcagaaagauuaagggcgcuucccgagguacacuauugccuggcgcagaaagacaaggaaacggcagccauugcu

SEQ ID NO: 153 - RNA, 1137 nt, Artificial Sequence
  Human GALT isoform 1
augucgcgcaguggaaccgauccucagcaacgccagcaggcgucagaggcggacgccgcagcagcaaccuuccgggcaaacgaccaucagcauauccgcuacaacccgcugcaggaugagugggugcuggugucagcucaccgcaugaagcggcccuggcagggucaaguggagccccagcuucugaagacagugccccgccaugacccucucaacccucuguguccuggggccauccgagccaacggagaggugaauccccaguacgauagcaccuuccuguuugacaacgacuucccagcucugcagccugaugcccccaguccaggacccagugaucauccccuuuuccaagcaaagucugcucgaggagucuguaaggucaugugcuuccaccccuggucggauguaacgcugccacucaugucggucccugagauccgggcuguuguugaugcaugggccucagucacagaggagcugggugcccaguacccuugggugcagaucuuugaaaacaaaggugccaugaugggcuguucuaacccccacccccacugccagguaugggccagcaguuuccugccagauauugcccagcgugaggagcgaucucagcaggccuauaagagucagcauggagagccccugcuaauggaguacagccgccaggagcuacucaggaaggaacgucugguccuaaccagugagcacugguuaguacugguccccuucugggcaacauggcccuaccagacacugcugcugccccgucggcaugugcggcggcuaccugagcugaccccugcugagcgugaugaucuagccuccaucaugaagaagcucuugaccaaguaugacaaccucuuugagacguccuuucccuacuccaugggcuggcauggggcucccacaggaucagaggcuggggccaacuggaaccauuggcagcugcacgcucauuacuacccuccgcuccugcgcucugccacuguccggaaauucaugguuggcuacgaaaugcuugcucaggcucagagggaccucaccccugagcaggcugcagagagacuaagggcacuuccugagguucauuaccaccuggggcagaaggacagggagacagcaaccaucgcc

SEQ ID NO: 154 - RNA, 1080 nt, Artificial Sequence
  Mouse GALT1  1-methyl-pseudouridine modified mRNA
auggcagcgaccuuccgggcgagcgaacaccagcauauucgcuacaacccgcuccaggacgaguggguguuagugucggcucaucgcaugaagcggcccuggcaaggacaaguggagccccagcuucugaagacagugccccgccacgacccacucaacccucugugucccggggccacacgagcuaauggggaggugaauccccacuaugaugguaccuuucuguuugacaaugacuucccggcucugcagcccgaugcuccggauccaggacccagugaccacccucucuuccgagcagaggccgccagaggaguuuguaaggucaugugcuuccaccccuggucggaugugacgcugccacucaugucugucccugagauccgagcugucaucgaugcaugggccucagucacagaggagcugggugcccaguacccuugggugcagaucuuugaaaauaaaggagccaugaugggcuguucuaacccccauccccacugccagguuugggcuagcagcuuccugccagauaucgcccagcgugaagagcgaucccagcagaccuaucacagccagcauggaaaaccuuuguuauuggaauauggucaccaagagcuccucaggaaggaacgucugguccuaaccagugagcacuggauaguucugguccccuucugggcaguguggccuuuccagacacuucugcugccccggcggcacgugcggcggcuaccugagcugaaccccgcugagcgugaugaucucgccuccaucaugaagaagcucuugaccaaguacgacaaucuauuugagacauccuuucccuacuccaugggcuggcauggggcucccacgggauuaaagacuggagccaccugugaccacuggcagcuccacgcccacuacuaccccccacuucugcgauccgcaacuguccggaaguucaugguuggcuaugaaaugcuugcccaggcccagcgugaccucacucccgaacaggccgcagaaagauuaagggcgcuucccgagguacacuauugccuggcgcagaaagacaaggaaacggcagccauugcu

SEQ ID NO: 155 - RNA, 85 nt, Artificial Sequence
  miR-126
cgcuggcgacgggacauuauuacuuuugguacgcgcugugacacuucaaacucguaccgugaguaauaaugcgccguccacggca

SEQ ID NO: 156 - RNA, 21 nt, Artificial Sequence
  miR-126-5p binding site
cgcguaccaaaaguaauaaug

SEQ ID NO: 157 - RNA, 69 nt, Artificial Sequence
  NTFIX ORF
augcuucuugccccuugggccuccccccagccccuccuccccuuccugcacccguacccccguggucuu

SEQ ID NO: 158 - RNA, 1303 nt, Artificial Sequence
  #20
gggaaauaagagagaaaagaagaguaagaagaaauauaagagccaccaugucgcgcaguggaaccgauccucagcaacgccagcaggcgucagaggcggacgccgcagcagcaaccuuccgggcaaacgaccaucagcauauccgcuacaacccgcugcaggaugagugggugcuggugucagcucaccgcaugaagcggcccuggcagggucaaguggagccccagcuucugaagacagugccccgccaugacccucucaacccucuguguccuggggccauccgagccaacggagaggugaauccccaguacgauagcaccuuccuguuugacaacgacuucccagcucugcagccugaugcccccaguccaggacccagugaucauccccuuuuccaagcaaagucugcucgaggagucuguaaggucaugugcuuccaccccuggucggauguaacgcugccacucaugucggucccugagauccgggcuguuguugaugcaugggccucagucacagaggagcugggugcccaguacccuugggugcagaucuuugaaaacaaaggugccaugaugggcuguucuaacccccacccccacugccagguaugggccagcaguuuccugccagauauugcccagcgugaggagcgaucucagcaggccuauaagagucagcauggagagccccugcuaauggaguacagccgccaggagcuacucaggaaggaacgucugguccuaaccagugagcacugguuaguacugguccccuucugggcaacauggcccuaccagacacugcugcugccccgucggcaugugcggcggcuaccugagcugaccccugcugagcgugaugaucuagccuccaucaugaagaagcucuugaccaaguaugacaaccucuuugagacguccuuucccuacuccaugggcuggcauggggcucccacaggaucagaggcuggggccaacuggaaccauuggcagcugcacgcucauuacuacccuccgcuccugcgcucugccacuguccggaaauucaugguuggcuacgaaaugcuugcucaggcucagagggaccucaccccugagcaggcugcagagagacuaagggcacuuccugagguucauuaccaccuggggcagaaggacagggagacagcaaccaucgccugauaauaggcuggagccucgguggccaugcuucuugccccuugggccuccccccagccccuccuccccuuccugcacccguacccccguggucuuugaauaaagucugagugggcggc

SEQ ID NO: 159 - RNA, 1127 nt, Artificial Sequence
  #21
gggaaauaagagagaaaagaagaguaagaagaaauauaagagccaccauggcagcgaccuuccgggcgagcgaacaccagcauauucgcuacaacccgcuccaggacgaguggguguuagugucggcucaucgcaugaagcggcccuggcaaggacaaguggagccccagcuucugaagacagugccccgccacgacccacucaacccucugugucccggggccacacgagcuaauggggaggugaauccccacuaugaugguaccuuucuguuugacaaugacuucccggcucugcagcccgaugcuccggauccaggacccagugaccacccucucuuccgagcagaggccgccagaggaguuuguaaggucaugugcuuccaccccuggucggaugugacgcugccacucaugucugucccugagauccgagcugucaucgaugcaugggccucagucacagaggagcugggugcccaguacccuugggugcagaucuuugaaaauaaaggagccaugaugggcuguucuaacccccauccccacugccagguuugggcuagcagcuuccugccagauaucgcccagcgugaagagcgaucccagcagaccuaucacagccagcauggaaaaccuuuguuauuggaauauggucaccaagagcuccucaggaaggaacgucugguccuaaccagugagcacuggauaguucugguccccuucugggcaguguggccuuuccagacacuucugcugccccggcggcacgugcggcggcuaccugagcugaaccccgcugagcgugaugaucucgccuccaucaugaagaagcucuugaccaaguacgacaaucuauuugagacauccuuucccuacuccaugggcuggcauggggcucccacgggauuaaagacuggagccaccugugaccacuggcagcuccacgcccacuacuaccccccacuucugcgauccgcaacuguccggaaguucaugguuggcuaugaaaugcuugcccaggcccagcgugaccucacucccgaacaggccgcagaaagauuaagggcgcuucccgagguacacuauugccuggcgcagaaagacaaggaaacggcagccauugcu

SEQ ID NO: 160 - RNA, 1363 nt, Artificial Sequence
  #22
gggaaauaagagagaaaagaagaguaagaagaaauauaagacagcgcgucaacauugccgaaucgccgggacucaucacaaucugccucuuggguuaucucuugucggcagauaccuucuuggaucacgaaaacgcgaacaaaauucuuaaucgcccgaagcgguauaacuccgggaaacuugaggaguuucagggcaaucuugaacgagacgaggagaacuccuuugaggaggcgagggaauuugaaaacacagagcgaacaacggaguuuuggaagcaauacguaggggaccagucgaauccccucaggggaucuaaagacaucaauagcuacugcccguuuggguuugaagggaagaacuagcugaccaacaucaaaaacggacgcuagcaguuuuguaagaacucggcugacaauaagguagucuccacagagggauaccggcuggcggagaaccaaaaauccgagcccgcagucccguucccuuggaggagcucacagacuagcaaguugacgagagcggagacuguauuccccgacgacuacgucaacagcaccgaagccgaaacaauccucgauaacaucacgcagagcacucaguccuucaacuuuacgagggucguagaggacgcgaaacccggucaguuccccuggcagguauugaacggaaaagucgccuuuugagguuccauugucaacgagaagauugucacagcggcacacugcguagaaacaggaaaaaucacgguagcgggagagcauaacauugaagagacagagcacacggaacaaaagcgaaucaucagaaucauuccacaccauaacuauaacgcggcaaucaauaaguacaaucacgacaucgcacuuuuggagcuugacgaaccuuugcuuaauucguacgucaccccuauuuguauugccgacaaagaguauacaaacaucuucuugaaauucggcuccggguacguaucgggcuggggcagauuccauaaggguagauccgcacuguugcaauaccucaggccccucgaucgagccacuugucugcgguccaccaaauucacaaucuacaacaauuucucgggauuccaagggagagauagcugccagggagacucaggggguccccacacggaagucgaggggacgucauuucugacgggaauuaucucgggagaggcgaaggggaacaucuacacuaaaucacgguucaauuggaucaaggaaaagacgaaacucacgugauaauaggcuggagccucgguggccaugcuucuugccccuugggccuccccccagccccuccuccccuuccugcacccguacccccguggucuuugaauaaagucugagugggcggc

SEQ ID NO: 161 - RNA, 976 nt, Artificial Sequence
  #23
gggaaauaagagagaaaagaagaguaagaagaaauauaagagccaccaugacccucucaacccucuguguccuggggccauccgagccaacggagaguaaggucaugugcuuccaccccuggucggauguaacgcugccacucaugucggucccugagauccgggcuguuguugaugcaugggccucagucacagaggagcugggugcccaguacccuugggugcagaucuuugaaaacaaaggugccaugaugggcuguucuaacccccacccccacugccagguaugggccagcaguuuccugccagauauugcccagcgugaggagcgaucucagcaggccuauaagagucagcauggagagccccugcuaauggaguacagccgccaggagcuacucaggaaggaacgucugguccuaaccagugagcacugguuaguacugguccccuucugggcaacauggcccuaccagacacugcugcugccccgucggcaugugcggcggcuaccugagcugaccccugcugagcgugaugaucuagccuccaucaugaagaagcucuugaccaaguaugacaaccucuuugagacguccuuucccuacuccaugggcuggcauggggcucccacaggaucagaggcuggggccaacuggaaccauuggcagcugcacgcucauuacuacccuccgcuccugcgcucugccacuguccggaaauucaugguuggcuacgaaaugcuugcucaggcucagagggaccucaccccugagcaggcugcagagagacuaagggcacuuccugagguucauuaccaccuggggcagaaggacagggagacagcaaccaucgccugauaauaggcuggagccucgguggccaugcuucuugccccuugggccuccccccagccccuccuccccuuccugcacccguacccccguggucuuugaauaaagucugagugggcggc

SEQ ID NO: 162 - RNA, 775 nt, Artificial Sequence
  #24
gggaaauaagagagaaaagaagaguaagaagaaauauaagagccaccaugaugggcuguucuaacccccauccccacugccagguuugggcuagcagcuuccugccagauaucgcccagcgugaagagcgaucccagcagaccuaucacagccagcauggaaaaccuuuguuauuggaauauggucaccaagagcuccucaggaaggaacgucugguccuaaccagugagcacuggauaguucugguccccuucugggcaguguggccuuuccagacacuucugcugccccggcggcacgugcggcggcuaccugagcugaaccccgcugagcgugaugaucucgccuccaucaugaagaagcucuugaccaaguacgacaaucuauuugagacauccuuucccuacuccaugggcuggcauggggcucccacgggauuaaagacuggagccaccugugaccacuggcagcuccacgcccacuacuaccccccacuucugcgauccgcaacuguccggaaguucaugguuggcuaugaaaugcuugcccaggcccagcgugaccucacucccgaacaggccgcagaaagauuaagggcgcuucccgagguacacuauugccuggcgcagaaagacaaggaaacggcagccauugcuugauaauaggcuggagccucgguggccaugcuucuugccccuugggccuccccccagccccuccuccccuuccugcacccguacccccguggucuuugaauaaagucugagugggcggc

SEQ ID NO: 163 - RNA, 164 nt, Artificial Sequence
  3' UTR (miR142+miR126 binding sites variant 2)
ugauaauaguccauaaaguaggaaacacuacagcuggagccucgguggccuagcuucuugccccuugggccuccccccagccccuccuccccuuccugcacccguaccccccgcauuauuacucacgguacgaguggucuuugaauaaagucugagugggcggc

SEQ ID NO: 164 - RNA, 142 nt, Artificial Sequence
  (3' UTR with miR 142-3p binding site variant 2)
ugauaauaggcuggagccucgguggccuagcuucuugccccuugggccuccccccagccccuccuccccuuccugcacccguacccccuccauaaaguaggaaacacuacaguggucuuugaauaaagucugagugggcggc

SEQ ID NO: 165 - RNA, 119 nt, Artificial Sequence
  (3' UTR, no miR binding sites variant 2)
ugauaauaggcuggagccucgguggccuagcuucuugccccuugggccuccccccagccccuccuccccuuccugcacccguacccccguggucuuugaauaaagucugagugggcggc

SEQ ID NO: 166 - RNA, 141 nt, Artificial Sequence
  (3' UTR with miR 126-3p binding site variant 3)
ugauaauaggcuggagccucgguggccuagcuucuugccccuugggccuccccccagccccuccuccccuuccugcacccguaccccccgcauuauuacucacgguacgaguggucuuugaauaaagucugagugggcggc

SEQ ID NO: 167 - RNA, 188 nt, Artificial Sequence
  (3' UTR with 3 miR 142-3p binding sites variant 2)
ugauaauaguccauaaaguaggaaacacuacagcuggagccucgguggccuagcuucuugccccuugggccuccauaaaguaggaaacacuacauccccccagccccuccuccccuuccugcacccguacccccuccauaaaguaggaaacacuacaguggucuuugaauaaagucugagugggcggc

SEQ ID NO: 168 - RNA, 142 nt, Artificial Sequence
  (3'UTR with miR 142-3p binding site, P1 insertion variant 2)
ugauaauaguccauaaaguaggaaacacuacagcuggagccucgguggccuagcuucuugccccuugggccuccccccagccccuccuccccuuccugcacccguacccccguggucuuugaauaaagucugagugggcggc

SEQ ID NO: 169 - RNA, 142 nt, Artificial Sequence
  (3'UTR with miR 142-3p binding site, P2 insertion variant 2)
ugauaauaggcuggagccucgguggcuccauaaaguaggaaacacuacacuagcuucuugccccuugggccuccccccagccccuccuccccuuccugcacccguacccccguggucuuugaauaaagucugagugggcggc

SEQ ID NO: 170 - RNA, 142 nt, Artificial Sequence
  (3'UTR with miR 142-3p binding site, P3 insertion variant 2)
ugauaauaggcuggagccucgguggccuagcuucuugccccuugggccuccauaaaguaggaaacacuacauccccccagccccuccuccccuuccugcacccguacccccguggucuuugaauaaagucugagugggcggc

SEQ ID NO: 171 - RNA, 142 nt, Artificial Sequence
  (3'UTR with miR 155-5p binding site variant 2)
ugauaauaggcuggagccucgguggccuagcuucuugccccuugggccuccccccagccccuccuccccuuccugcacccguacccccaccccuaucacaauuagcauuaaguggucuuugaauaaagucugagugggcggc

SEQ ID NO: 172 - RNA, 188 nt, Artificial Sequence
  (3' UTR with 3 miR 155-5p binding sites variant 2)
ugauaauagaccccuaucacaauuagcauuaagcuggagccucgguggccuagcuucuugccccuugggccaccccuaucacaauuagcauuaauccccccagccccuccuccccuuccugcacccguacccccaccccuaucacaauuagcauuaaguggucuuugaauaaagucugagugggcggc

SEQ ID NO: 173 - RNA, 188 nt, Artificial Sequence
  (3'UTR with 2 miR 155-5p binding sites and 1 miR 142-3p binding site variant 2)
ugauaauagaccccuaucacaauuagcauuaagcuggagccucgguggccuagcuucuugccccuugggccuccauaaaguaggaaacacuacauccccccagccccuccuccccuuccugcacccguacccccaccccuaucacaauuagcauuaaguggucuuugaauaaagucugagugggcggc